European Patent Application EP 4 389 759 A1, published June 26, 2024. Title: ISOLATED MODIFIED AAV5 CAPSID PROTEIN VP1. Applicant: Joint Stock Company «BIOCAD». Application WO PCT/RU2022/050257, filed August 21, 2022. The sequence listing filed with the application follows.

SEQUENCE LISTING (48 sequences)

SEQ ID NO: 1 - protein, 724 aa, Adeno-associated dependoparvovirus B
MSFVDHPPDWLEEVGEGLREFLGLEAGPPKPKPNQQHQDQARGLVLPGYNYLGPGNGLDRGEPVNRADEVAREHDISYNEQLEAGDNPYLKYNHADAEFQEKLADDTSFGGNLGKAVFQAKKRVLEPFGLVEEGAKTAPTGKRIDDHFPKRKKARTEEDSKPSTSSDAEAGPSGSQQLQIPAQPASSLGADTMSAGGGGPLGDNNQGADGVGNASGDWHCDSTWMGDRVVTKSTRTWVLPSYNNHQYREIKSGSVDGSNANAYFGYSTPWGYFDFNRFHSHWSPRDWQRLINNYWGFRPRSLRVKIFNIQVKEVTVQDSTTTIANNLTSTVQVFTDDDYQLPYVVGNGTEGCLPAFPPQVFTLPQYGYATLNRDNTENPTERSSFFCLEYFPSKMLRTGNNFEFTYNFEEVPFHSSFAPSQNLFKLANPLVDQYLYRFVSTNNTGGVQFNKNLAGRYANTYKNWFPGPMGRTQGWNLGSGVNRASVSAFATTNRMELEGASYQVPPQPNGMTNNLQGSNTYALENTMIFNSQPANPGTTATYLEGNMLITSESETQPVNRVAYNVGGQMATNNQSSTTAPATGTYNLQEIVPGSVWMERDVYLQGPIWAKIPETGAHFHPSPAMGGFGLKHPPPMMLIKNTPVPGNITSFSDVPVSSFITQYSTGQVTVEMEWELKKENSKRWNPEIQYTNNYNDPQFVDFAPDSTGEYRTTRPIGTRYLTRPL

SEQ ID NO: 2 - protein, 724 aa, synthetic construct
MAFVDHPPDWLEEVGEGLREFLGLEAGPPKPKPNQQHQDQARGLVLPGYNYLGPGNGLDRGEPVNRADEVAREHDISYNEQLEAGDNPYLKYNHADAEFQEKLADDTSFGGNLGKAVFQAKKRVLEPFGLVEEGAKTAPTGKRIDDHFPKRKKARTEEDSKPSTSSDAEAGPSGSQQLQIPAQPASSLGADTMSAGGGGPLGDNNQGADGVGNASGDWHCDSTWMGDRVVTKSTRTWVLPSYNNHQYREIKSGSVDGSNANAYFGYSTPWGYFDFNRFHSHWSPRDWQRLINNYWGFRPRSLRVKIFNIQVKEVTVQDSTTTIANNLTSTVQVFTDDDYQLPYVVGNGTEGCLPAFPPQVFTLPQYGYATLNRDNTENPTERSSFFCLEYFPSKMLRTGNNFEFTYNFEEVPFHSSFAPSQNLFKLANPLVDQYLYRFVSTNNTGGVQFNKNLAGRYANTYKNWFPGPMGRTQGWNLGSGVNRASVSAFATTNRMELEGASYQVPPQPNGMTNNLQGSNTYALENTMIFNSQPANPGTTATYLEGNMLITSESETQPVNRVAYNVGGQMATNNQSSTTAPATGTYNLQEIVPGSVWMERDVYLQGPIWAKIPETGAHFHPSPAMGGFGLKHPPPMMLIKNTPVPGNITSFSDVPVSSFITQYSTGQVTVEMEWELKKENSKRWNPEIQYTNNYNDPQFVDFAPDSTGEYRSTRPIGTRYLTRPL

SEQ ID NO: 3 - protein, 724 aa, synthetic construct
MSFVDHPPDWLEEVGEGLREFLGLEAGPPKPKPNQQHQDQARGLVLPGYNYLGPGNGLDRGEPVNRADEVAREHDISYNEQLEAGDNPYLKYNHADAEFQEKLADDTSFGGNLGKAVFQAKKRVLEPFGLVEEGAKTAPTGKRIDDHFPKRKKARTEEDSKPSTSSDAEAGPSGSQQLQIPAQPASSLGADTMSAGGGGPLGDNNQGADGVGNASGDWHCDSTWMVDRVVTKSTRTWVLPSYNNHQYREIKSGSVDGSNANAYFGYSTPWGYFDFNRFHSHWSPRDWQRLINNYWGFRPRSLRVKIFNIQVKEVTVQDSTTTIANNLTSTVQVFTDDDYQLPYVVGNGTEGCLPAFPPQVFTLPQYGYATLNRDNTENPTERSSFFCLEYFPSKMLRTGNNFEFTYNFEEVPFHSSFAPSQNLFKLANPLVDQYLYRFVSTNNTGGVQFNKNLAGRYANTYKNWFPGPMGRTQGWNLGSGVNRASVSAFATTNRMELEGASYQVPPQPNGMTNNLQGSNTYALENTMIFNSQPANPGTTATYLEGNMLITSESETQPVNRVAYNVGGQMATNNQSSTTAPATGTYNLQEIVPGSVWMERDVYLQGPIWAKIPETGAHFHPSPAMGGFGLKHPPPMMLIKNTPVPGNITSFSDVPVSSFITQYSTGQVTVEMEWELKKENSKRWNPEIQYTNNYNDPQFVDFAPDSTGEYRTTRPIGTRYLTRPL

SEQ ID NO: 4 - protein, 724 aa, synthetic construct
MAFVDHPPDWLEEVGEGLREFLGLEAGPPKPKPNQQHQDQARGLVLPGYNYLGPGNGLDRGEPVNRADEVAREHDISYNEQLEAGDNPYLKYNHADAEFQEKLADDTSFGGNLGKAVFQAKKRVLEPFGLVEEGAKTAPTGKRIDDHFPKRKKARTEEDSKPSTSSDAEAGPSGSQQLQIPAQPASSLGADTMSAGGGGPLGDNNQGADGVGNASGDWHCDSTWMVDRVVTKSTRTWVLPSYNNHQYREIKSGSVDGSNANAYFGYSTPWGYFDFNRFHSHWSPRDWQRLINNYWGFRPRSLRVKIFNIQVKEVTVQDSTTTIANNLTSTVQVFTDDDYQLPYVVGNGTEGCLPAFPPQVFTLPQYGYATLNRDNTENPTERSSFFCLEYFPSKMLRTGNNFEFTYNFEEVPFHSSFAPSQNLFKLANPLVDQYLYRFVSTNNTGGVQFNKNLAGRYANTYKNWFPGPMGRTQGWNLGSGVNRASVSAFATTNRMELEGASYQVPPQPNGMTNNLQGSNTYALENTMIFNSQPANPGTTATYLEGNMLITSESETQPVNRVAYNVGGQMATNNQSSTTAPATGTYNLQEIVPGSVWMERDVYLQGPIWAKIPETGAHFHPSPAMGGFGLKHPPPMMLIKNTPVPGNITSFSDVPVSSFITQYSTGQVTVEMEWELKKENSKRWNPEIQYTNNYNDPQFVDFAPDSTGEYRSTRPIGTRYLTRPL

SEQ ID NO: 5 - protein, 724 aa, synthetic construct
MSFVDHPPDWLEEVGEGLREFLGLEAGPPKPKPNQQHQDQARGLVLPGYNYLGPGNGLDRGEPVNRADEVAREHDISYNEQLEAGDNPYLKYNHADAEFQEKLADDTSFGGNLGKAVFQAKKRVLEPFGLVEEGAKTAPTGKRIDDHFPKRKKARTEEDSKPSTSSDAEAGPSGSQQLQIPAQPASSLGADTMSAGGGGPLGDNNQGADGVGNASGDWHCDSTWMGDRVVTKSTRTWVLPSYNNHQYREIKSGSVDGSNANAYFGYSTPWGYFDFNRFHSHWSPRDWQRLINNYWGFRPRSLRVKIFNIQVKEVTVQDSTTTIANNLTSTVQVFTDDDYQLPYVVGNGTEGCLPAFPPQVFTLPQYGYATLNRDNTENPTERSSFFCLEYFPSKMLRTGNNFEFTYNFEEVPFHSSFAPSQNLFKLANPLVDQYLYRFVSTNNTGGVQFNKNLAGRYANTYKNWFPGPMGRTQGWNLGSGVNRASVSAFATTNRMELEGASYQVPPQPNGMTNNLQGSNTYALENTMIFNSQPANPGTTATYLEGNMLITSESETQPVNRVAYNVGGQMATNNQSSTTAPATGTYNLQEIVPGSVWMERDVYLQGPIWAKIPEAGAHFHPSPAMGGFGLKHPPPMMLIKNTPVPGNITSFSDVPVSSFITQYSTGQVTVEMEWELKKENSKRWNPEIQYTNNYNDPQFVDFAPDSTGEYRTTRPIGTRYLTRPL

SEQ ID NO: 6 - protein, 724 aa, synthetic construct
MAFVDHPPDWLEEVGEGLREFLGLEAGPPKPKPNQQHQDQARGLVLPGYNYLGPGNGLDRGEPVNRADEVAREHDISYNEQLEAGDNPYLKYNHADAEFQEKLADDTSFGGNLGKAVFQAKKRVLEPFGLVEEGAKTAPTGKRIDDHFPKRKKARTEEDSKPSTSSDAEAGPSGSQQLQIPAQPASSLGADTMSAGGGGPLGDNNQGADGVGNASGDWHCDSTWMGDRVVTKSTRTWVLPSYNNHQYREIKSGSVDGSNANAYFGYSTPWGYFDFNRFHSHWSPRDWQRLINNYWGFRPRSLRVKIFNIQVKEVTVQDSTTTIANNLTSTVQVFTDDDYQLPYVVGNGTEGCLPAFPPQVFTLPQYGYATLNRDNTENPTERSSFFCLEYFPSKMLRTGNNFEFTYNFEEVPFHSSFAPSQNLFKLANPLVDQYLYRFVSTNNTGGVQFNKNLAGRYANTYKNWFPGPMGRTQGWNLGSGVNRASVSAFATTNRMELEGASYQVPPQPNGMTNNLQGSNTYALENTMIFNSQPANPGTTATYLEGNMLITSESETQPVNRVAYNVGGQMATNNQSSTTAPATGTYNLQEIVPGSVWMERDVYLQGPIWAKIPEAGAHFHPSPAMGGFGLKHPPPMMLIKNTPVPGNITSFSDVPVSSFITQYSTGQVTVEMEWELKKENSKRWNPEIQYTNNYNDPQFVDFAPDSTGEYRSTRPIGTRYLTRPL

SEQ ID NO: 7 - protein, 724 aa, synthetic construct
MSFVDHPPDWLEEVGEGLREFLGLEAGPPKPKPNQQHQDQARGLVLPGYNYLGPGNGLDRGEPVNRADEVAREHDISYNEQLEAGDNPYLKYNHADAEFQEKLADDTSFGGNLGKAVFQAKKRVLEPFGLVEEGAKTAPTGKRIDDHFPKRKKARTEEDSKPSTSSDAEAGPSGSQQLQIPAQPASSLGADTMSAGGGGPLGDNNQGADGVGNASGDWHCDSTWMGDRVVTKSTRTWVLPSYNNHQYREIKSGSVDGSNANAYFGYSTPWGYFDFNRFHSHWSPRDWQRLINNYWGFRPRSLRVKIFNIQVKEVTVQDSTTTIANNLTSTVQVFTDDDYQLPYVVGNGTEGCLPAFPPQVFTLPQYGYATLNRDNTENPTERSSFFCLEYFPSKMLRTGNNFEFTYNFEEVPFHSSFAPSQNLFKLANPLVDQYLYRFVSTNNTGGVQFNKNLAGRYANTYKNWFPGPMGRTQGWNLGSGVNRASVSAFATTNRMELEGASYQVPPQPNGMTNNLQGSNTYALENTMIFNSQPANPGTTATYLEGNMLITSESETQPVNRVAYNVGGQMATNNQSSTTAPATGTYNLQEIVPGSVWMERDVYLQGPIWAKIPEVGAHFHPSPAMGGFGLKHPPPMMLIKNTPVPGNITSFSDVPVSSFITQYSTGQVTVEMEWELKKENSKRWNPEIQYTNNYNDPQFVDFAPDSTGEYRTTRPIGTRYLTRPL

SEQ ID NO: 8 - protein, 724 aa, synthetic construct
MAFVDHPPDWLEEVGEGLREFLGLEAGPPKPKPNQQHQDQARGLVLPGYNYLGPGNGLDRGEPVNRADEVAREHDISYNEQLEAGDNPYLKYNHADAEFQEKLADDTSFGGNLGKAVFQAKKRVLEPFGLVEEGAKTAPTGKRIDDHFPKRKKARTEEDSKPSTSSDAEAGPSGSQQLQIPAQPASSLGADTMSAGGGGPLGDNNQGADGVGNASGDWHCDSTWMGDRVVTKSTRTWVLPSYNNHQYREIKSGSVDGSNANAYFGYSTPWGYFDFNRFHSHWSPRDWQRLINNYWGFRPRSLRVKIFNIQVKEVTVQDSTTTIANNLTSTVQVFTDDDYQLPYVVGNGTEGCLPAFPPQVFTLPQYGYATLNRDNTENPTERSSFFCLEYFPSKMLRTGNNFEFTYNFEEVPFHSSFAPSQNLFKLANPLVDQYLYRFVSTNNTGGVQFNKNLAGRYANTYKNWFPGPMGRTQGWNLGSGVNRASVSAFATTNRMELEGASYQVPPQPNGMTNNLQGSNTYALENTMIFNSQPANPGTTATYLEGNMLITSESETQPVNRVAYNVGGQMATNNQSSTTAPATGTYNLQEIVPGSVWMERDVYLQGPIWAKIPEVGAHFHPSPAMGGFGLKHPPPMMLIKNTPVPGNITSFSDVPVSSFITQYSTGQVTVEMEWELKKENSKRWNPEIQYTNNYNDPQFVDFAPDSTGEYRSTRPIGTRYLTRPL

SEQ ID NO: 9 - DNA, 2175 bp, Adeno-associated dependoparvovirus B
  source 1..2175: mol_type = genomic DNA
atgtcttttgttgatcaccctccagattggttggaagaagttggtgaaggtcttcgcgagtttttgggccttgaagcgggcccaccgaaaccaaaacccaatcagcagcatcaagatcaagcccgtggtcttgtgctgcctggttataactatctcggacccggaaacggtctcgatcgaggagagcctgtcaacagggcagacgaggtcgcgcgagagcacgacatctcgtacaacgagcagcttgaggcgggagacaacccctacctcaagtacaaccacgcggacgccgagtttcaggagaagctcgccgacgacacatccttcgggggaaacctcggaaaggcagtctttcaggccaagaaaagggttctcgaaccttttggcctggttgaagagggtgctaagacggcccctaccggaaagcggatagacgaccactttccaaaaagaaagaaggctcggaccgaagaggactccaagccttccacctcgtcagacgccgaagctggacccagcggatcccagcagctgcaaatcccagcccaaccagcctcaagtttgggagctgatacaatgtctgcgggaggtggcggcccattgggcgacaataaccaaggtgccgatggagtgggcaatgcctcgggagattggcattgcgattccacgtggatgggggacagagtcgtcaccaagtccacccgaacctgggtgctgcccagctacaacaaccaccagtaccgagagatcaaaagcggctccgtcgacggaagcaacgccaacgcctactttggatacagcaccccctgggggtactttgactttaaccgcttccacagccactggagcccccgagactggcaaagactcatcaacaactactggggcttcagaccccggtccctcagagtcaaaatcttcaacattcaagtcaaagaggtcacggtgcaggactccaccaccaccatcgccaacaacctcacctccaccgtccaagtgtttacggacgacgactaccagctgccctacgtcgtcggcaacgggaccgagggatgcctgccggccttccctccgcaggtctttacgctgccgcagtacggttacgcgacgctgaaccgcgacaacacagaaaatcccaccgagaggagcagcttcttctgcctagagtactttcccagcaagatgctgagaacgggcaacaactttgagtttacctacaactttgaggaggtgcccttccactccagcttcgctcccagtcagaacctcttcaagctggccaacccgctggtggaccagtacttgtaccgcttcgtgagcacaaataacactggcggagtccagttcaacaagaacctggccgggagatacgccaacacctacaaaaactggttcccggggcccatgggccgaacccagggctggaacctgggctccggggtcaaccgcgccagtgtcagcgccttcgccacgaccaataggatggagctcgagggcgcgagttaccaggtgcccccgcagccgaacggcatgaccaacaacctccagggcagcaacacctatgccctggagaacactatgatcttcaacagccagccggcgaacccgggcaccaccgccacgtacctcgagggcaacatgctcatcaccagcgagagcgagacgcagccggtgaaccgcgtggcgtacaacgtcggcgggcagatggccaccaacaaccagagctccaccactgcccccgcgaccggcacgtacaacctccaggaaatcgtgcccggcagcgtgtggatggagagggacgtgtacctccaaggacccatctgggccaagatcccagagacgggggcgcactttcacccctctccggccatgggcggattcggactcaaacacccaccgcccatgatgctcatcaagaacacgcctgtgcccggaaatatcaccagcttctcggacgtgcccgtcagcagcttcatcacccagtacagcaccgggcaggtcaccgtggagatggagtgggagctcaagaaggaaaactccaagaggtggaacccagagatccagtacacaaacaactacaacgacccccagtttgtggactttgccccggacagcaccggggaatacagaaccaccagacctatcggaacccgataccttacccgacccctttaa

SEQ ID NO: 10 - DNA, 2175 bp, synthetic construct
  source 1..2175: mol_type = other DNA
atggcttttgttgatcaccctccagattggttggaagaagttggtgaaggtcttcgcgagtttttgggccttgaagcgggcccaccgaaaccaaaacccaatcagcagcatcaagatcaagcccgtggtcttgtgctgcctggttataactatctcggacccggaaacggtctcgatcgaggagagcctgtcaacagggcagacgaggtcgcgcgagagcacgacatctcgtacaacgagcagcttgaggcgggagacaacccctacctcaagtacaaccacgcggacgccgagtttcaggagaagctcgccgacgacacatccttcgggggaaacctcggaaaggcagtctttcaggccaagaaaagggttctcgaaccttttggcctggttgaagagggtgctaagacggcccctaccggaaagcggatagacgaccactttccaaaaagaaagaaggctcggaccgaagaggactccaagccttccacctcgtcagacgccgaagctggacccagcggatcccagcagctgcaaatcccagcccaaccagcctcaagtttgggagctgatacaatgtctgcgggaggtggcggcccattgggcgacaataaccaaggtgccgatggagtgggcaatgcctcgggagattggcattgcgattccacgtggatgggggacagagtcgtcaccaagtccacccgaacctgggtgctgcccagctacaacaaccaccagtaccgagagatcaaaagcggctccgtcgacggaagcaacgccaacgcctactttggatacagcaccccctgggggtactttgactttaaccgcttccacagccactggagcccccgagactggcaaagactcatcaacaactactggggcttcagaccccggtccctcagagtcaaaatcttcaacattcaagtcaaagaggtcacggtgcaggactccaccaccaccatcgccaacaacctcacctccaccgtccaagtgtttacggacgacgactaccagctgccctacgtcgtcggcaacgggaccgagggatgcctgccggccttccctccgcaggtctttacgctgccgcagtacggttacgcgacgctgaaccgcgacaacacagaaaatcccaccgagaggagcagcttcttctgcctagagtactttcccagcaagatgctgagaacgggcaacaactttgagtttacctacaactttgaggaggtgcccttccactccagcttcgctcccagtcagaacctcttcaagctggccaacccgctggtggaccagtacttgtaccgcttcgtgagcacaaataacactggcggagtccagttcaacaagaacctggccgggagatacgccaacacctacaaaaactggttcccggggcccatgggccgaacccagggctggaacctgggctccggggtcaaccgcgccagtgtcagcgccttcgccacgaccaataggatggagctcgagggcgcgagttaccaggtgcccccgcagccgaacggcatgaccaacaacctccagggcagcaacacctatgccctggagaacactatgatcttcaacagccagccggcgaacccgggcaccaccgccacgtacctcgagggcaacatgctcatcaccagcgagagcgagacgcagccggtgaaccgcgtggcgtacaacgtcggcgggcagatggccaccaacaaccagagctccaccactgcccccgcgaccggcacgtacaacctccaggaaatcgtgcccggcagcgtgtggatggagagggacgtgtacctccaaggacccatctgggccaagatcccagagacgggggcgcactttcacccctctccggccatgggcggattcggactcaaacacccaccgcccatgatgctcatcaagaacacgcctgtgcccggaaatatcaccagcttctcggacgtgcccgtcagcagcttcatcacccagtacagcaccgggcaggtcaccgtggagatggagtgggagctcaagaaggaaaactccaagaggtggaacccagagatccagtacacaaacaactacaacgacccccagtttgtggactttgccccggacagcaccggggaatacagaagcaccagacctatcggaacccgataccttacccgacccctttaa

SEQ ID NO: 11 - DNA, 2175 bp, synthetic construct
  source 1..2175: mol_type = other DNA
atgtcttttgttgatcaccctccagattggttggaagaagttggtgaaggtcttcgcgagtttttgggccttgaagcgggcccaccgaaaccaaaacccaatcagcagcatcaagatcaagcccgtggtcttgtgctgcctggttataactatctcggacccggaaacggtctcgatcgaggagagcctgtcaacagggcagacgaggtcgcgcgagagcacgacatctcgtacaacgagcagcttgaggcgggagacaacccctacctcaagtacaaccacgcggacgccgagtttcaggagaagctcgccgacgacacatccttcgggggaaacctcggaaaggcagtctttcaggccaagaaaagggttctcgaaccttttggcctggttgaagagggtgctaagacggcccctaccggaaagcggatagacgaccactttccaaaaagaaagaaggctcggaccgaagaggactccaagccttccacctcgtcagacgccgaagctggacccagcggatcccagcagctgcaaatcccagcccaaccagcctcaagtttgggagctgatacaatgtctgcgggaggtggcggcccattgggcgacaataaccaaggtgccgatggagtgggcaatgcctcgggagattggcattgcgattccacgtggatggtcgacagagtcgtcaccaagtccacccgaacctgggtgctgcccagctacaacaaccaccagtaccgagagatcaaaagcggctccgtcgacggaagcaacgccaacgcctactttggatacagcaccccctgggggtactttgactttaaccgcttccacagccactggagcccccgagactggcaaagactcatcaacaactactggggcttcagaccccggtccctcagagtcaaaatcttcaacattcaagtcaaagaggtcacggtgcaggactccaccaccaccatcgccaacaacctcacctccaccgtccaagtgtttacggacgacgactaccagctgccctacgtcgtcggcaacgggaccgagggatgcctgccggccttccctccgcaggtctttacgctgccgcagtacggttacgcgacgctgaaccgcgacaacacagaaaatcccaccgagaggagcagcttcttctgcctagagtactttcccagcaagatgctgagaacgggcaacaactttgagtttacctacaactttgaggaggtgcccttccactccagcttcgctcccagtcagaacctcttcaagctggccaacccgctggtggaccagtacttgtaccgcttcgtgagcacaaataacactggcggagtccagttcaacaagaacctggccgggagatacgccaacacctacaaaaactggttcccggggcccatgggccgaacccagggctggaacctgggctccggggtcaaccgcgccagtgtcagcgccttcgccacgaccaataggatggagctcgagggcgcgagttaccaggtgcccccgcagccgaacggcatgaccaacaacctccagggcagcaacacctatgccctggagaacactatgatcttcaacagccagccggcgaacccgggcaccaccgccacgtacctcgagggcaacatgctcatcaccagcgagagcgagacgcagccggtgaaccgcgtggcgtacaacgtcggcgggcagatggccaccaacaaccagagctccaccactgcccccgcgaccggcacgtacaacctccaggaaatcgtgcccggcagcgtgtggatggagagggacgtgtacctccaaggacccatctgggccaagatcccagagacgggggcgcactttcacccctctccggccatgggcggattcggactcaaacacccaccgcccatgatgctcatcaagaacacgcctgtgcccggaaatatcaccagcttctcggacgtgcccgtcagcagcttcatcacccagtacagcaccgggcaggtcaccgtggagatggagtgggagctcaagaaggaaaactccaagaggtggaacccagagatccagtacacaaacaactacaacgacccccagtttgtggactttgccccggacagcaccggggaatacagaaccaccagacctatcggaacccgataccttacccgacccctttaa

SEQ ID NO: 12 - DNA, 2175 bp, synthetic construct
  source 1..2175: mol_type = other DNA
atggcttttgttgatcaccctccagattggttggaagaagttggtgaaggtcttcgcgagtttttgggccttgaagcgggcccaccgaaaccaaaacccaatcagcagcatcaagatcaagcccgtggtcttgtgctgcctggttataactatctcggacccggaaacggtctcgatcgaggagagcctgtcaacagggcagacgaggtcgcgcgagagcacgacatctcgtacaacgagcagcttgaggcgggagacaacccctacctcaagtacaaccacgcggacgccgagtttcaggagaagctcgccgacgacacatccttcgggggaaacctcggaaaggcagtctttcaggccaagaaaagggttctcgaaccttttggcctggttgaagagggtgctaagacggcccctaccggaaagcggatagacgaccactttccaaaaagaaagaaggctcggaccgaagaggactccaagccttccacctcgtcagacgccgaagctggacccagcggatcccagcagctgcaaatcccagcccaaccagcctcaagtttgggagctgatacaatgtctgcgggaggtggcggcccattgggcgacaataaccaaggtgccgatggagtgggcaatgcctcgggagattggcattgcgattccacgtggatggtcgacagagtcgtcaccaagtccacccgaacctgggtgctgcccagctacaacaaccaccagtaccgagagatcaaaagcggctccgtcgacggaagcaacgccaacgcctactttggatacagcaccccctgggggtactttgactttaaccgcttccacagccactggagcccccgagactggcaaagactcatcaacaactactggggcttcagaccccggtccctcagagtcaaaatcttcaacattcaagtcaaagaggtcacggtgcaggactccaccaccaccatcgccaacaacctcacctccaccgtccaagtgtttacggacgacgactaccagctgccctacgtcgtcggcaacgggaccgagggatgcctgccggccttccctccgcaggtctttacgctgccgcagtacggttacgcgacgctgaaccgcgacaacacagaaaatcccaccgagaggagcagcttcttctgcctagagtactttcccagcaagatgctgagaacgggcaacaactttgagtttacctacaactttgaggaggtgcccttccactccagcttcgctcccagtcagaacctcttcaagctggccaacccgctggtggaccagtacttgtaccgcttcgtgagcacaaataacactggcggagtccagttcaacaagaacctggccgggagatacgccaacacctacaaaaactggttcccggggcccatgggccgaacccagggctggaacctgggctccggggtcaaccgcgccagtgtcagcgccttcgccacgaccaataggatggagctcgagggcgcgagttaccaggtgcccccgcagccgaacggcatgaccaacaacctccagggcagcaacacctatgccctggagaacactatgatcttcaacagccagccggcgaacccgggcaccaccgccacgtacctcgagggcaacatgctcatcaccagcgagagcgagacgcagccggtgaaccgcgtggcgtacaacgtcggcgggcagatggccaccaacaaccagagctccaccactgcccccgcgaccggcacgtacaacctccaggaaatcgtgcccggcagcgtgtggatggagagggacgtgtacctccaaggacccatctgggccaagatcccagagacgggggcgcactttcacccctctccggccatgggcggattcggactcaaacacccaccgcccatgatgctcatcaagaacacgcctgtgcccggaaatatcaccagcttctcggacgtgcccgtcagcagcttcatcacccagtacagcaccgggcaggtcaccgtggagatggagtgggagctcaagaaggaaaactccaagaggtggaacccagagatccagtacacaaacaactacaacgacccccagtttgtggactttgccccggacagcaccggggaatacagaagcaccagacctatcggaacccgataccttacccgacccctttaa

SEQ ID NO: 13 - DNA, 2175 bp, synthetic construct
  source 1..2175: mol_type = other DNA
atgtcttttgttgatcaccctccagattggttggaagaagttggtgaaggtcttcgcgagtttttgggccttgaagcgggcccaccgaaaccaaaacccaatcagcagcatcaagatcaagcccgtggtcttgtgctgcctggttataactatctcggacccggaaacggtctcgatcgaggagagcctgtcaacagggcagacgaggtcgcgcgagagcacgacatctcgtacaacgagcagcttgaggcgggagacaacccctacctcaagtacaaccacgcggacgccgagtttcaggagaagctcgccgacgacacatccttcgggggaaacctcggaaaggcagtctttcaggccaagaaaagggttctcgaaccttttggcctggttgaagagggtgctaagacggcccctaccggaaagcggatagacgaccactttccaaaaagaaagaaggctcggaccgaagaggactccaagccttccacctcgtcagacgccgaagctggacccagcggatcccagcagctgcaaatcccagcccaaccagcctcaagtttgggagctgatacaatgtctgcgggaggtggcggcccattgggcgacaataaccaaggtgccgatggagtgggcaatgcctcgggagattggcattgcgattccacgtggatgggggacagagtcgtcaccaagtccacccgaacctgggtgctgcccagctacaacaaccaccagtaccgagagatcaaaagcggctccgtcgacggaagcaacgccaacgcctactttggatacagcaccccctgggggtactttgactttaaccgcttccacagccactggagcccccgagactggcaaagactcatcaacaactactggggcttcagaccccggtccctcagagtcaaaatcttcaacattcaagtcaaagaggtcacggtgcaggactccaccaccaccatcgccaacaacctcacctccaccgtccaagtgtttacggacgacgactaccagctgccctacgtcgtcggcaacgggaccgagggatgcctgccggccttccctccgcaggtctttacgctgccgcagtacggttacgcgacgctgaaccgcgacaacacagaaaatcccaccgagaggagcagcttcttctgcctagagtactttcccagcaagatgctgagaacgggcaacaactttgagtttacctacaactttgaggaggtgcccttccactccagcttcgctcccagtcagaacctcttcaagctggccaacccgctggtggaccagtacttgtaccgcttcgtgagcacaaataacactggcggagtccagttcaacaagaacctggccgggagatacgccaacacctacaaaaactggttcccggggcccatgggccgaacccagggctggaacctgggctccggggtcaaccgcgccagtgtcagcgccttcgccacgaccaataggatggagctcgagggcgcgagttaccaggtgcccccgcagccgaacggcatgaccaacaacctccagggcagcaacacctatgccctggagaacactatgatcttcaacagccagccggcgaacccgggcaccaccgccacgtacctcgagggcaacatgctcatcaccagcgagagcgagacgcagccggtgaaccgcgtggcgtacaacgtcggcgggcagatggccaccaacaaccagagctccaccactgcccccgcgaccggcacgtacaacctccaggaaatcgtgcccggcagcgtgtggatggagagggacgtgtacctccaaggacccatctgggccaagatcccagaggccggggcgcactttcacccctctccggccatgggcggattcggactcaaacacccaccgcccatgatgctcatcaagaacacgcctgtgcccggaaatatcaccagcttctcggacgtgcccgtcagcagcttcatcacccagtacagcaccgggcaggtcaccgtggagatggagtgggagctcaagaaggaaaactccaagaggtggaacccagagatccagtacacaaacaactacaacgacccccagtttgtggactttgccccggacagcaccggggaatacagaaccaccagacctatcggaacccgataccttacccgacccctttaa

SEQ ID NO: 14 - DNA, 2175 bp, synthetic construct
  source 1..2175: mol_type = other DNA
atggcttttgttgatcaccctccagattggttggaagaagttggtgaaggtcttcgcgagtttttgggccttgaagcgggcccaccgaaaccaaaacccaatcagcagcatcaagatcaagcccgtggtcttgtgctgcctggttataactatctcggacccggaaacggtctcgatcgaggagagcctgtcaacagggcagacgaggtcgcgcgagagcacgacatctcgtacaacgagcagcttgaggcgggagacaacccctacctcaagtacaaccacgcggacgccgagtttcaggagaagctcgccgacgacacatccttcgggggaaacctcggaaaggcagtctttcaggccaagaaaagggttctcgaaccttttggcctggttgaagagggtgctaagacggcccctaccggaaagcggatagacgaccactttccaaaaagaaagaaggctcggaccgaagaggactccaagccttccacctcgtcagacgccgaagctggacccagcggatcccagcagctgcaaatcccagcccaaccagcctcaagtttgggagctgatacaatgtctgcgggaggtggcggcccattgggcgacaataaccaaggtgccgatggagtgggcaatgcctcgggagattggcattgcgattccacgtggatgggggacagagtcgtcaccaagtccacccgaacctgggtgctgcccagctacaacaaccaccagtaccgagagatcaaaagcggctccgtcgacggaagcaacgccaacgcctactttggatacagcaccccctgggggtactttgactttaaccgcttccacagccactggagcccccgagactggcaaagactcatcaacaactactggggcttcagaccccggtccctcagagtcaaaatcttcaacattcaagtcaaagaggtcacggtgcaggactccaccaccaccatcgccaacaacctcacctccaccgtccaagtgtttacggacgacgactaccagctgccctacgtcgtcggcaacgggaccgagggatgcctgccggccttccctccgcaggtctttacgctgccgcagtacggttacgcgacgctgaaccgcgacaacacagaaaatcccaccgagaggagcagcttcttctgcctagagtactttcccagcaagatgctgagaacgggcaacaactttgagtttacctacaactttgaggaggtgcccttccactccagcttcgctcccagtcagaacctcttcaagctggccaacccgctggtggaccagtacttgtaccgcttcgtgagcacaaataacactggcggagtccagttcaacaagaacctggccgggagatacgccaacacctacaaaaactggttcccggggcccatgggccgaacccagggctggaacctgggctccggggtcaaccgcgccagtgtcagcgccttcgccacgaccaataggatggagctcgagggcgcgagttaccaggtgcccccgcagccgaacggcatgaccaacaacctccagggcagcaacacctatgccctggagaacactatgatcttcaacagccagccggcgaacccgggcaccaccgccacgtacctcgagggcaacatgctcatcaccagcgagagcgagacgcagccggtgaaccgcgtggcgtacaacgtcggcgggcagatggccaccaacaaccagagctccaccactgcccccgcgaccggcacgtacaacctccaggaaatcgtgcccggcagcgtgtggatggagagggacgtgtacctccaaggacccatctgggccaagatcccagaggccggggcgcactttcacccctctccggccatgggcggattcggactcaaacacccaccgcccatgatgctcatcaagaacacgcctgtgcccggaaatatcaccagcttctcggacgtgcccgtcagcagcttcatcacccagtacagcaccgggcaggtcaccgtggagatggagtgggagctcaagaaggaaaactccaagaggtggaacccagagatccagtacacaaacaactacaacgacccccagtttgtggactttgccccggacagcaccggggaatacagaagcaccagacctatcggaacccgataccttacccgacccctttaa

SEQ ID NO: 15 - DNA, 2175 bp, synthetic construct
  source 1..2175: mol_type = other DNA
atgtcttttgttgatcaccctccagattggttggaagaagttggtgaaggtcttcgcgagtttttgggccttgaagcgggcccaccgaaaccaaaacccaatcagcagcatcaagatcaagcccgtggtcttgtgctgcctggttataactatctcggacccggaaacggtctcgatcgaggagagcctgtcaacagggcagacgaggtcgcgcgagagcacgacatctcgtacaacgagcagcttgaggcgggagacaacccctacctcaagtacaaccacgcggacgccgagtttcaggagaagctcgccgacgacacatccttcgggggaaacctcggaaaggcagtctttcaggccaagaaaagggttctcgaaccttttggcctggttgaagagggtgctaagacggcccctaccggaaagcggatagacgaccactttccaaaaagaaagaaggctcggaccgaagaggactccaagccttccacctcgtcagacgccgaagctggacccagcggatcccagcagctgcaaatcccagcccaaccagcctcaagtttgggagctgatacaatgtctgcgggaggtggcggcccattgggcgacaataaccaaggtgccgatggagtgggcaatgcctcgggagattggcattgcgattccacgtggatgggggacagagtcgtcaccaagtccacccgaacctgggtgctgcccagctacaacaaccaccagtaccgagagatcaaaagcggctccgtcgacggaagcaacgccaacgcctactttggatacagcaccccctgggggtactttgactttaaccgcttccacagccactggagcccccgagactggcaaagactcatcaacaactactggggcttcagaccccggtccctcagagtcaaaatcttcaacattcaagtcaaagaggtcacggtgcaggactccaccaccaccatcgccaacaacctcacctccaccgtccaagtgtttacggacgacgactaccagctgccctacgtcgtcggcaacgggaccgagggatgcctgccggccttccctccgcaggtctttacgctgccgcagtacggttacgcgacgctgaaccgcgacaacacagaaaatcccaccgagaggagcagcttcttctgcctagagtactttcccagcaagatgctgagaacgggcaacaactttgagtttacctacaactttgaggaggtgcccttccactccagcttcgctcccagtcagaacctcttcaagctggccaacccgctggtggaccagtacttgtaccgcttcgtgagcacaaataacactggcggagtccagttcaacaagaacctggccgggagatacgccaacacctacaaaaactggttcccggggcccatgggccgaacccagggctggaacctgggctccggggtcaaccgcgccagtgtcagcgccttcgccacgaccaataggatggagctcgagggcgcgagttaccaggtgcccccgcagccgaacggcatgaccaacaacctccagggcagcaacacctatgccctggagaacactatgatcttcaacagccagccggcgaacccgggcaccaccgccacgtacctcgagggcaacatgctcatcaccagcgagagcgagacgcagccggtgaaccgcgtggcgtacaacgtcggcgggcagatggccaccaacaaccagagctccaccactgcccccgcgaccggcacgtacaacctccaggaaatcgtgcccggcagcgtgtggatggagagggacgtgtacctccaaggacccatctgggccaagatcccagaggtcggggcgcactttcacccctctccggccatgggcggattcggactcaaacacccaccgcccatgatgctcatcaagaacacgcctgtgcccggaaatatcaccagcttctcggacgtgcccgtcagcagcttcatcacccagtacagcaccgggcaggtcaccgtggagatggagtgggagctcaagaaggaaaactccaagaggtggaacccagagatccagtacacaaacaactacaacgacccccagtttgtggactttgccccggacagcaccggggaatacagaaccaccagacctatcggaacccgataccttacccgacccctttaa

SEQ ID NO: 16 - DNA, 2175 bp, synthetic construct
  source 1..2175: mol_type = other DNA
atggcttttgttgatcaccctccagattggttggaagaagttggtgaaggtcttcgcgagtttttgggccttgaagcgggcccaccgaaaccaaaacccaatcagcagcatcaagatcaagcccgtggtcttgtgctgcctggttataactatctcggacccggaaacggtctcgatcgaggagagcctgtcaacagggcagacgaggtcgcgcgagagcacgacatctcgtacaacgagcagcttgaggcgggagacaacccctacctcaagtacaaccacgcggacgccgagtttcaggagaagctcgccgacgacacatccttcgggggaaacctcggaaaggcagtctttcaggccaagaaaagggttctcgaaccttttggcctggttgaagagggtgctaagacggcccctaccggaaagcggatagacgaccactttccaaaaagaaagaaggctcggaccgaagaggactccaagccttccacctcgtcagacgccgaagctggacccagcggatcccagcagctgcaaatcccagcccaaccagcctcaagtttgggagctgatacaatgtctgcgggaggtggcggcccattgggcgacaataaccaaggtgccgatggagtgggcaatgcctcgggagattggcattgcgattccacgtggatgggggacagagtcgtcaccaagtccacccgaacctgggtgctgcccagctacaacaaccaccagtaccgagagatcaaaagcggctccgtcgacggaagcaacgccaacgcctactttggatacagcaccccctgggggtactttgactttaaccgcttccacagccactggagcccccgagactggcaaagactcatcaacaactactggggcttcagaccccggtccctcagagtcaaaatcttcaacattcaagtcaaagaggtcacggtgcaggactccaccaccaccatcgccaacaacctcacctccaccgtccaagtgtttacggacgacgactaccagctgccctacgtcgtcggcaacgggaccgagggatgcctgccggccttccctccgcaggtctttacgctgccgcagtacggttacgcgacgctgaaccgcgacaacacagaaaatcccaccgagaggagcagcttcttctgcctagagtactttcccagcaagatgctgagaacgggcaacaactttgagtttacctacaactttgaggaggtgcccttccactccagcttcgctcccagtcagaacctcttcaagctggccaacccgctggtggaccagtacttgtaccgcttcgtgagcacaaataacactggcggagtccagttcaacaagaacctggccgggagatacgccaacacctacaaaaactggttcccggggcccatgggccgaacccagggctggaacctgggctccggggtcaaccgcgccagtgtcagcgccttcgccacgaccaataggatggagctcgagggcgcgagttaccaggtgcccccgcagccgaacggcatgaccaacaacctccagggcagcaacacctatgccctggagaacactatgatcttcaacagccagccggcgaacccgggcaccaccgccacgtacctcgagggcaacatgctcatcaccagcgagagcgagacgcagccggtgaaccgcgtggcgtacaacgtcggcgggcagatggccaccaacaaccagagctccaccactgcccccgcgaccggcacgtacaacctccaggaaatcgtgcccggcagcgtgtggatggagagggacgtgtacctccaaggacccatctgggccaagatcccagaggtcggggcgcactttcacccctctccggccatgggcggattcggactcaaacacccaccgcccatgatgctcatcaagaacacgcctgtgcccggaaatatcaccagcttctcggacgtgcccgtcagcagcttcatcacccagtacagcaccgggcaggtcaccgtggagatggagtgggagctcaagaaggaaaactccaagaggtggaacccagagatccagtacacaaacaactacaacgacccccagtttgtggactttgccccggacagcaccggggaatacagaagcaccagacctatcggaacccgataccttacccgacccctttaa

SEQ ID NO: 17 - protein, 588 aa, Adeno-associated dependoparvovirus B
TAPTGKRIDDHFPKRKKARTEEDSKPSTSSDAEAGPSGSQQLQIPAQPASSLGADTMSAGGGGPLGDNNQGADGVGNASGDWHCDSTWMGDRVVTKSTRTWVLPSYNNHQYREIKSGSVDGSNANAYFGYSTPWGYFDFNRFHSHWSPRDWQRLINNYWGFRPRSLRVKIFNIQVKEVTVQDSTTTIANNLTSTVQVFTDDDYQLPYVVGNGTEGCLPAFPPQVFTLPQYGYATLNRDNTENPTERSSFFCLEYFPSKMLRTGNNFEFTYNFEEVPFHSSFAPSQNLFKLANPLVDQYLYRFVSTNNTGGVQFNKNLAGRYANTYKNWFPGPMGRTQGWNLGSGVNRASVSAFATTNRMELEGASYQVPPQPNGMTNNLQGSNTYALENTMIFNSQPANPGTTATYLEGNMLITSESETQPVNRVAYNVGGQMATNNQSSTTAPATGTYNLQEIVPGSVWMERDVYLQGPIWAKIPETGAHFHPSPAMGGFGLKHPPPMMLIKNTPVPGNITSFSDVPVSSFITQYSTGQVTVEMEWELKKENSKRWNPEIQYTNNYNDPQFVDFAPDSTGEYRTTRPIGTRYLTRPL

SEQ ID NO: 18 - protein, 588 aa, synthetic construct
TAPTGKRIDDHFPKRKKARTEEDSKPSTSSDAEAGPSGSQQLQIPAQPASSLGADTMSAGGGGPLGDNNQGADGVGNASGDWHCDSTWMGDRVVTKSTRTWVLPSYNNHQYREIKSGSVDGSNANAYFGYSTPWGYFDFNRFHSHWSPRDWQRLINNYWGFRPRSLRVKIFNIQVKEVTVQDSTTTIANNLTSTVQVFTDDDYQLPYVVGNGTEGCLPAFPPQVFTLPQYGYATLNRDNTENPTERSSFFCLEYFPSKMLRTGNNFEFTYNFEEVPFHSSFAPSQNLFKLANPLVDQYLYRFVSTNNTGGVQFNKNLAGRYANTYKNWFPGPMGRTQGWNLGSGVNRASVSAFATTNRMELEGASYQVPPQPNGMTNNLQGSNTYALENTMIFNSQPANPGTTATYLEGNMLITSESETQPVNRVAYNVGGQMATNNQSSTTAPATGTYNLQEIVPGSVWMERDVYLQGPIWAKIPETGAHFHPSPAMGGFGLKHPPPMMLIKNTPVPGNITSFSDVPVSSFITQYSTGQVTVEMEWELKKENSKRWNPEIQYTNNYNDPQFVDFAPDSTGEYRSTRPIGTRYLTRPL

SEQ ID NO: 19 - protein, 588 aa, synthetic construct
TAPTGKRIDDHFPKRKKARTEEDSKPSTSSDAEAGPSGSQQLQIPAQPASSLGADTMSAGGGGPLGDNNQGADGVGNASGDWHCDSTWMVDRVVTKSTRTWVLPSYNNHQYREIKSGSVDGSNANAYFGYSTPWGYFDFNRFHSHWSPRDWQRLINNYWGFRPRSLRVKIFNIQVKEVTVQDSTTTIANNLTSTVQVFTDDDYQLPYVVGNGTEGCLPAFPPQVFTLPQYGYATLNRDNTENPTERSSFFCLEYFPSKMLRTGNNFEFTYNFEEVPFHSSFAPSQNLFKLANPLVDQYLYRFVSTNNTGGVQFNKNLAGRYANTYKNWFPGPMGRTQGWNLGSGVNRASVSAFATTNRMELEGASYQVPPQPNGMTNNLQGSNTYALENTMIFNSQPANPGTTATYLEGNMLITSESETQPVNRVAYNVGGQMATNNQSSTTAPATGTYNLQEIVPGSVWMERDVYLQGPIWAKIPETGAHFHPSPAMGGFGLKHPPPMMLIKNTPVPGNITSFSDVPVSSFITQYSTGQVTVEMEWELKKENSKRWNPEIQYTNNYNDPQFVDFAPDSTGEYRTTRPIGTRYLTRPL

SEQ ID NO: 20 - protein, 588 aa, synthetic construct
TAPTGKRIDDHFPKRKKARTEEDSKPSTSSDAEAGPSGSQQLQIPAQPASSLGADTMSAGGGGPLGDNNQGADGVGNASGDWHCDSTWMVDRVVTKSTRTWVLPSYNNHQYREIKSGSVDGSNANAYFGYSTPWGYFDFNRFHSHWSPRDWQRLINNYWGFRPRSLRVKIFNIQVKEVTVQDSTTTIANNLTSTVQVFTDDDYQLPYVVGNGTEGCLPAFPPQVFTLPQYGYATLNRDNTENPTERSSFFCLEYFPSKMLRTGNNFEFTYNFEEVPFHSSFAPSQNLFKLANPLVDQYLYRFVSTNNTGGVQFNKNLAGRYANTYKNWFPGPMGRTQGWNLGSGVNRASVSAFATTNRMELEGASYQVPPQPNGMTNNLQGSNTYALENTMIFNSQPANPGTTATYLEGNMLITSESETQPVNRVAYNVGGQMATNNQSSTTAPATGTYNLQEIVPGSVWMERDVYLQGPIWAKIPETGAHFHPSPAMGGFGLKHPPPMMLIKNTPVPGNITSFSDVPVSSFITQYSTGQVTVEMEWELKKENSKRWNPEIQYTNNYNDPQFVDFAPDSTGEYRSTRPIGTRYLTRPL

SEQ ID NO: 21 - protein, 588 aa, synthetic construct
TAPTGKRIDDHFPKRKKARTEEDSKPSTSSDAEAGPSGSQQLQIPAQPASSLGADTMSAGGGGPLGDNNQGADGVGNASGDWHCDSTWMGDRVVTKSTRTWVLPSYNNHQYREIKSGSVDGSNANAYFGYSTPWGYFDFNRFHSHWSPRDWQRLINNYWGFRPRSLRVKIFNIQVKEVTVQDSTTTIANNLTSTVQVFTDDDYQLPYVVGNGTEGCLPAFPPQVFTLPQYGYATLNRDNTENPTERSSFFCLEYFPSKMLRTGNNFEFTYNFEEVPFHSSFAPSQNLFKLANPLVDQYLYRFVSTNNTGGVQFNKNLAGRYANTYKNWFPGPMGRTQGWNLGSGVNRASVSAFATTNRMELEGASYQVPPQPNGMTNNLQGSNTYALENTMIFNSQPANPGTTATYLEGNMLITSESETQPVNRVAYNVGGQMATNNQSSTTAPATGTYNLQEIVPGSVWMERDVYLQGPIWAKIPEAGAHFHPSPAMGGFGLKHPPPMMLIKNTPVPGNITSFSDVPVSSFITQYSTGQVTVEMEWELKKENSKRWNPEIQYTNNYNDPQFVDFAPDSTGEYRTTRPIGTRYLTRPL

SEQ ID NO: 22 - protein, 588 aa, synthetic construct
TAPTGKRIDDHFPKRKKARTEEDSKPSTSSDAEAGPSGSQQLQIPAQPASSLGADTMSAGGGGPLGDNNQGADGVGNASGDWHCDSTWMGDRVVTKSTRTWVLPSYNNHQYREIKSGSVDGSNANAYFGYSTPWGYFDFNRFHSHWSPRDWQRLINNYWGFRPRSLRVKIFNIQVKEVTVQDSTTTIANNLTSTVQVFTDDDYQLPYVVGNGTEGCLPAFPPQVFTLPQYGYATLNRDNTENPTERSSFFCLEYFPSKMLRTGNNFEFTYNFEEVPFHSSFAPSQNLFKLANPLVDQYLYRFVSTNNTGGVQFNKNLAGRYANTYKNWFPGPMGRTQGWNLGSGVNRASVSAFATTNRMELEGASYQVPPQPNGMTNNLQGSNTYALENTMIFNSQPANPGTTATYLEGNMLITSESETQPVNRVAYNVGGQMATNNQSSTTAPATGTYNLQEIVPGSVWMERDVYLQGPIWAKIPEAGAHFHPSPAMGGFGLKHPPPMMLIKNTPVPGNITSFSDVPVSSFITQYSTGQVTVEMEWELKKENSKRWNPEIQYTNNYNDPQFVDFAPDSTGEYRSTRPIGTRYLTRPL

SEQ ID NO: 23 - protein, 588 aa, synthetic construct
TAPTGKRIDDHFPKRKKARTEEDSKPSTSSDAEAGPSGSQQLQIPAQPASSLGADTMSAGGGGPLGDNNQGADGVGNASGDWHCDSTWMGDRVVTKSTRTWVLPSYNNHQYREIKSGSVDGSNANAYFGYSTPWGYFDFNRFHSHWSPRDWQRLINNYWGFRPRSLRVKIFNIQVKEVTVQDSTTTIANNLTSTVQVFTDDDYQLPYVVGNGTEGCLPAFPPQVFTLPQYGYATLNRDNTENPTERSSFFCLEYFPSKMLRTGNNFEFTYNFEEVPFHSSFAPSQNLFKLANPLVDQYLYRFVSTNNTGGVQFNKNLAGRYANTYKNWFPGPMGRTQGWNLGSGVNRASVSAFATTNRMELEGASYQVPPQPNGMTNNLQGSNTYALENTMIFNSQPANPGTTATYLEGNMLITSESETQPVNRVAYNVGGQMATNNQSSTTAPATGTYNLQEIVPGSVWMERDVYLQGPIWAKIPEVGAHFHPSPAMGGFGLKHPPPMMLIKNTPVPGNITSFSDVPVSSFITQYSTGQVTVEMEWELKKENSKRWNPEIQYTNNYNDPQFVDFAPDSTGEYRTTRPIGTRYLTRPL

SEQ ID NO: 24 - protein, 588 aa, synthetic construct
TAPTGKRIDDHFPKRKKARTEEDSKPSTSSDAEAGPSGSQQLQIPAQPASSLGADTMSAGGGGPLGDNNQGADGVGNASGDWHCDSTWMGDRVVTKSTRTWVLPSYNNHQYREIKSGSVDGSNANAYFGYSTPWGYFDFNRFHSHWSPRDWQRLINNYWGFRPRSLRVKIFNIQVKEVTVQDSTTTIANNLTSTVQVFTDDDYQLPYVVGNGTEGCLPAFPPQVFTLPQYGYATLNRDNTENPTERSSFFCLEYFPSKMLRTGNNFEFTYNFEEVPFHSSFAPSQNLFKLANPLVDQYLYRFVSTNNTGGVQFNKNLAGRYANTYKNWFPGPMGRTQGWNLGSGVNRASVSAFATTNRMELEGASYQVPPQPNGMTNNLQGSNTYALENTMIFNSQPANPGTTATYLEGNMLITSESETQPVNRVAYNVGGQMATNNQSSTTAPATGTYNLQEIVPGSVWMERDVYLQGPIWAKIPEVGAHFHPSPAMGGFGLKHPPPMMLIKNTPVPGNITSFSDVPVSSFITQYSTGQVTVEMEWELKKENSKRWNPEIQYTNNYNDPQFVDFAPDSTGEYRSTRPIGTRYLTRPL

SEQ ID NO: 25 - DNA, 1767 bp, Adeno-associated dependoparvovirus B
  source 1..1767: mol_type = genomic DNA
acggcccctaccggaaagcggatagacgaccactttccaaaaagaaagaaggctcggaccgaagaggactccaagccttccacctcgtcagacgccgaagctggacccagcggatcccagcagctgcaaatcccagcccaaccagcctcaagtttgggagctgatacaatgtctgcgggaggtggcggcccattgggcgacaataaccaaggtgccgatggagtgggcaatgcctcgggagattggcattgcgattccacgtggatgggggacagagtcgtcaccaagtccacccgaacctgggtgctgcccagctacaacaaccaccagtaccgagagatcaaaagcggctccgtcgacggaagcaacgccaacgcctactttggatacagcaccccctgggggtactttgactttaaccgcttccacagccactggagcccccgagactggcaaagactcatcaacaactactggggcttcagaccccggtccctcagagtcaaaatcttcaacattcaagtcaaagaggtcacggtgcaggactccaccaccaccatcgccaacaacctcacctccaccgtccaagtgtttacggacgacgactaccagctgccctacgtcgtcggcaacgggaccgagggatgcctgccggccttccctccgcaggtctttacgctgccgcagtacggttacgcgacgctgaaccgcgacaacacagaaaatcccaccgagaggagcagcttcttctgcctagagtactttcccagcaagatgctgagaacgggcaacaactttgagtttacctacaactttgaggaggtgcccttccactccagcttcgctcccagtcagaacctcttcaagctggccaacccgctggtggaccagtacttgtaccgcttcgtgagcacaaataacactggcggagtccagttcaacaagaacctggccgggagatacgccaacacctacaaaaactggttcccggggcccatgggccgaacccagggctggaacctgggctccggggtcaaccgcgccagtgtcagcgccttcgccacgaccaataggatggagctcgagggcgcgagttaccaggtgcccccgcagccgaacggcatgaccaacaacctccagggcagcaacacctatgccctggagaacactatgatcttcaacagccagccggcgaacccgggcaccaccgccacgtacctcgagggcaacatgctcatcaccagcgagagcgagacgcagccggtgaaccgcgtggcgtacaacgtcggcgggcagatggccaccaacaaccagagctccaccactgcccccgcgaccggcacgtacaacctccaggaaatcgtgcccggcagcgtgtggatggagagggacgtgtacctccaaggacccatctgggccaagatcccagagacgggggcgcactttcacccctctccggccatgggcggattcggactcaaacacccaccgcccatgatgctcatcaagaacacgcctgtgcccggaaatatcaccagcttctcggacgtgcccgtcagcagcttcatcacccagtacagcaccgggcaggtcaccgtggagatggagtgggagctcaagaaggaaaactccaagaggtggaacccagagatccagtacacaaacaactacaacgacccccagtttgtggactttgccccggacagcaccggggaatacagaaccaccagacctatcggaacccgataccttacccgacccctttaa

SEQ ID NO: 26 - DNA, 1767 bp, synthetic construct
  source 1..1767: mol_type = other DNA
acggcccctaccggaaagcggatagacgaccactttccaaaaagaaagaaggctcggaccgaagaggactccaagccttccacctcgtcagacgccgaagctggacccagcggatcccagcagctgcaaatcccagcccaaccagcctcaagtttgggagctgatacaatgtctgcgggaggtggcggcccattgggcgacaataaccaaggtgccgatggagtgggcaatgcctcgggagattggcattgcgattccacgtggatgggggacagagtcgtcaccaagtccacccgaacctgggtgctgcccagctacaacaaccaccagtaccgagagatcaaaagcggctccgtcgacggaagcaacgccaacgcctactttggatacagcaccccctgggggtactttgactttaaccgcttccacagccactggagcccccgagactggcaaagactcatcaacaactactggggcttcagaccccggtccctcagagtcaaaatcttcaacattcaagtcaaagaggtcacggtgcaggactccaccaccaccatcgccaacaacctcacctccaccgtccaagtgtttacggacgacgactaccagctgccctacgtcgtcggcaacgggaccgagggatgcctgccggccttccctccgcaggtctttacgctgccgcagtacggttacgcgacgctgaaccgcgacaacacagaaaatcccaccgagaggagcagcttcttctgcctagagtactttcccagcaagatgctgagaacgggcaacaactttgagtttacctacaactttgaggaggtgcccttccactccagcttcgctcccagtcagaacctcttcaagctggccaacccgctggtggaccagtacttgtaccgcttcgtgagcacaaataacactggcggagtccagttcaacaagaacctggccgggagatacgccaacacctacaaaaactggttcccggggcccatgggccgaacccagggctggaacctgggctccggggtcaaccgcgccagtgtcagcgccttcgccacgaccaataggatggagctcgagggcgcgagttaccaggtgcccccgcagccgaacggcatgaccaacaacctccagggcagcaacacctatgccctggagaacactatgatcttcaacagccagccggcgaacccgggcaccaccgccacgtacctcgagggcaacatgctcatcaccagcgagagcgagacgcagccggtgaaccgcgtggcgtacaacgtcggcgggcagatggccaccaacaaccagagctccaccactgcccccgcgaccggcacgtacaacctccaggaaatcgtgcccggcagcgtgtggatggagagggacgtgtacctccaaggacccatctgggccaagatcccagagacgggggcgcactttcacccctctccggccatgggcggattcggactcaaacacccaccgcccatgatgctcatcaagaacacgcctgtgcccggaaatatcaccagcttctcggacgtgcccgtcagcagcttcatcacccagtacagcaccgggcaggtcaccgtggagatggagtgggagctcaagaaggaaaactccaagaggtggaacccagagatccagtacacaaacaactacaacgacccccagtttgtggactttgccccggacagcaccggggaatacagaagcaccagacctatcggaacccgataccttacccgacccctttaa

SEQ ID NO: 27 - DNA, 1767 bp, synthetic construct
  source 1..1767: mol_type = other DNA
acggcccctaccggaaagcggatagacgaccactttccaaaaagaaagaaggctcggaccgaagaggactccaagccttccacctcgtcagacgccgaagctggacccagcggatcccagcagctgcaaatcccagcccaaccagcctcaagtttgggagctgatacaatgtctgcgggaggtggcggcccattgggcgacaataaccaaggtgccgatggagtgggcaatgcctcgggagattggcattgcgattccacgtggatggtcgacagagtcgtcaccaagtccacccgaacctgggtgctgcccagctacaacaaccaccagtaccgagagatcaaaagcggctccgtcgacggaagcaacgccaacgcctactttggatacagcaccccctgggggtactttgactttaaccgcttccacagccactggagcccccgagactggcaaagactcatcaacaactactggggcttcagaccccggtccctcagagtcaaaatcttcaacattcaagtcaaagaggtcacggtgcaggactccaccaccaccatcgccaacaacctcacctccaccgtccaagtgtttacggacgacgactaccagctgccctacgtcgtcggcaacgggaccgagggatgcctgccggccttccctccgcaggtctttacgctgccgcagtacggttacgcgacgctgaaccgcgacaacacagaaaatcccaccgagaggagcagcttcttctgcctagagtactttcccagcaagatgctgagaacgggcaacaactttgagtttacctacaactttgaggaggtgcccttccactccagcttcgctcccagtcagaacctcttcaagctggccaacccgctggtggaccagtacttgtaccgcttcgtgagcacaaataacactggcggagtccagttcaacaagaacctggccgggagatacgccaacacctacaaaaactggttcccggggcccatgggccgaacccagggctggaacctgggctccggggtcaaccgcgccagtgtcagcgccttcgccacgaccaataggatggagctcgagggcgcgagttaccaggtgcccccgcagccgaacggcatgaccaacaacctccagggcagcaacacctatgccctggagaacactatgatcttcaacagccagccggcgaacccgggcaccaccgccacgtacctcgagggcaacatgctcatcaccagcgagagcgagacgcagccggtgaaccgcgtggcgtacaacgtcggcgggcagatggccaccaacaaccagagctccaccactgcccccgcgaccggcacgtacaacctccaggaaatcgtgcccggcagcgtgtggatggagagggacgtgtacctccaaggacccatctgggccaagatcccagagacgggggcgcactttcacccctctccggccatgggcggattcggactcaaacacccaccgcccatgatgctcatcaagaacacgcctgtgcccggaaatatcaccagcttctcggacgtgcccgtcagcagcttcatcacccagtacagcaccgggcaggtcaccgtggagatggagtgggagctcaagaaggaaaactccaagaggtggaacccagagatccagtacacaaacaactacaacgacccccagtttgtggactttgccccggacagcaccggggaatacagaaccaccagacctatcggaacccgataccttacccgacccctttaa

SEQ ID NO: 28 - DNA, 1767 bp, synthetic construct
  source 1..1767: mol_type = other DNA
acggcccctaccggaaagcggatagacgaccactttccaaaaagaaagaaggctcggaccgaagaggactccaagccttccacctcgtcagacgccgaagctggacccagcggatcccagcagctgcaaatcccagcccaaccagcctcaagtttgggagctgatacaatgtctgcgggaggtggcggcccattgggcgacaataaccaaggtgccgatggagtgggcaatgcctcgggagattggcattgcgattccacgtggatggtcgacagagtcgtcaccaagtccacccgaacctgggtgctgcccagctacaacaaccaccagtaccgagagatcaaaagcggctccgtcgacggaagcaacgccaacgcctactttggatacagcaccccctgggggtactttgactttaaccgcttccacagccactggagcccccgagactggcaaagactcatcaacaactactggggcttcagaccccggtccctcagagtcaaaatcttcaacattcaagtcaaagaggtcacggtgcaggactccaccaccaccatcgccaacaacctcacctccaccgtccaagtgtttacggacgacgactaccagctgccctacgtcgtcggcaacgggaccgagggatgcctgccggccttccctccgcaggtctttacgctgccgcagtacggttacgcgacgctgaaccgcgacaacacagaaaatcccaccgagaggagcagcttcttctgcctagagtactttcccagcaagatgctgagaacgggcaacaactttgagtttacctacaactttgaggaggtgcccttccactccagcttcgctcccagtcagaacctcttcaagctggccaacccgctggtggaccagtacttgtaccgcttcgtgagcacaaataacactggcggagtccagttcaacaagaacctggccgggagatacgccaacacctacaaaaactggttcccggggcccatgggccgaacccagggctggaacctgggctccggggtcaaccgcgccagtgtcagcgccttcgccacgaccaataggatggagctcgagggcgcgagttaccaggtgcccccgcagccgaacggcatgaccaacaacctccagggcagcaacacctatgccctggagaacactatgatcttcaacagccagccggcgaacccgggcaccaccgccacgtacctcgagggcaacatgctcatcaccagcgagagcgagacgcagccggtgaaccgcgtggcgtacaacgtcggcgggcagatggccaccaacaaccagagctccaccactgcccccgcgaccggcacgtacaacctccaggaaatcgtgcccggcagcgtgtggatggagagggacgtgtacctccaaggacccatctgggccaagatcccagagacgggggcgcactttcacccctctccggccatgggcggattcggactcaaacacccaccgcccatgatgctcatcaagaacacgcctgtgcccggaaatatcaccagcttctcggacgtgcccgtcagcagcttcatcacccagtacagcaccgggcaggtcaccgtggagatggagtgggagctcaagaaggaaaactccaagaggtggaacccagagatccagtacacaaacaactacaacgacccccagtttgtggactttgccccggacagcaccggggaatacagaagcaccagacctatcggaacccgataccttacccgacccctttaa

SEQ ID NO: 29 - DNA, 1767 bp, synthetic construct
  source 1..1767: mol_type = other DNA
acggcccctaccggaaagcggatagacgaccactttccaaaaagaaagaaggctcggaccgaagaggactccaagccttccacctcgtcagacgccgaagctggacccagcggatcccagcagctgcaaatcccagcccaaccagcctcaagtttgggagctgatacaatgtctgcgggaggtggcggcccattgggcgacaataaccaaggtgccgatggagtgggcaatgcctcgggagattggcattgcgattccacgtggatgggggacagagtcgtcaccaagtccacccgaacctgggtgctgcccagctacaacaaccaccagtaccgagagatcaaaagcggctccgtcgacggaagcaacgccaacgcctactttggatacagcaccccctgggggtactttgactttaaccgcttccacagccactggagcccccgagactggcaaagactcatcaacaactactggggcttcagaccccggtccctcagagtcaaaatcttcaacattcaagtcaaagaggtcacggtgcaggactccaccaccaccatcgccaacaacctcacctccaccgtccaagtgtttacggacgacgactaccagctgccctacgtcgtcggcaacgggaccgagggatgcctgccggccttccctccgcaggtctttacgctgccgcagtacggttacgcgacgctgaaccgcgacaacacagaaaatcccaccgagaggagcagcttcttctgcctagagtactttcccagcaagatgctgagaacgggcaacaactttgagtttacctacaactttgaggaggtgcccttccactccagcttcgctcccagtcagaacctcttcaagctggccaacccgctggtggaccagtacttgtaccgcttcgtgagcacaaataacactggcggagtccagttcaacaagaacctggccgggagatacgccaacacctacaaaaactggttcccggggcccatgggccgaacccagggctggaacctgggctccggggtcaaccgcgccagtgtcagcgccttcgccacgaccaataggatggagctcgagggcgcgagttaccaggtgcccccgcagccgaacggcatgaccaacaacctccagggcagcaacacctatgccctggagaacactatgatcttcaacagccagccggcgaacccgggcaccaccgccacgtacctcgagggcaacatgctcatcaccagcgagagcgagacgcagccggtgaaccgcgtggcgtacaacgtcggcgggcagatggccaccaacaaccagagctccaccactgcccccgcgaccggcacgtacaacctccaggaaatcgtgcccggcagcgtgtggatggagagggacgtgtacctccaaggacccatctgggccaagatcccagaggccggggcgcactttcacccctctccggccatgggcggattcggactcaaacacccaccgcccatgatgctcatcaagaacacgcctgtgcccggaaatatcaccagcttctcggacgtgcccgtcagcagcttcatcacccagtacagcaccgggcaggtcaccgtggagatggagtgggagctcaagaaggaaaactccaagaggtggaacccagagatccagtacacaaacaactacaacgacccccagtttgtggactttgccccggacagcaccggggaatacagaaccaccagacctatcggaacccgataccttacccgacccctttaa

SEQ ID NO: 30 - DNA, 1767 bp, synthetic construct
  source 1..1767: mol_type = other DNA
acggcccctaccggaaagcggatagacgaccactttccaaaaagaaagaaggctcggaccgaagaggactccaagccttccacctcgtcagacgccgaagctggacccagcggatcccagcagctgcaaatcccagcccaaccagcctcaagtttgggagctgatacaatgtctgcgggaggtggcggcccattgggcgacaataaccaaggtgccgatggagtgggcaatgcctcgggagattggcattgcgattccacgtggatgggggacagagtcgtcaccaagtccacccgaacctgggtgctgcccagctacaacaaccaccagtaccgagagatcaaaagcggctccgtcgacggaagcaacgccaacgcctactttggatacagcaccccctgggggtactttgactttaaccgcttccacagccactggagcccccgagactggcaaagactcatcaacaactactggggcttcagaccccggtccctcagagtcaaaatcttcaacattcaagtcaaagaggtcacggtgcaggactccaccaccaccatcgccaacaacctcacctccaccgtccaagtgtttacggacgacgactaccagctgccctacgtcgtcggcaacgggaccgagggatgcctgccggccttccctccgcaggtctttacgctgccgcagtacggttacgcgacgctgaaccgcgacaacacagaaaatcccaccgagaggagcagcttcttctgcctagagtactttcccagcaagatgctgagaacgggcaacaactttgagtttacctacaactttgaggaggtgcccttccactccagcttcgctcccagtcagaacctcttcaagctggccaacccgctggtggaccagtacttgtaccgcttcgtgagcacaaataacactggcggagtccagttcaacaagaacctggccgggagatacgccaacacctacaaaaactggttcccggggcccatgggccgaacccagggctggaacctgggctccggggtcaaccgcgccagtgtcagcgccttcgccacgaccaataggatggagctcgagggcgcgagttaccaggtgcccccgcagccgaacggcatgaccaacaacctccagggcagcaacacctatgccctggagaacactatgatcttcaacagccagccggcgaacccgggcaccaccgccacgtacctcgagggcaacatgctcatcaccagcgagagcgagacgcagccggtgaaccgcgtggcgtacaacgtcggcgggcagatggccaccaacaaccagagctccaccactgcccccgcgaccggcacgtacaacctccaggaaatcgtgcccggcagcgtgtggatggagagggacgtgtacctccaaggacccatctgggccaagatcccagaggccggggcgcactttcacccctctccggccatgggcggattcggactcaaacacccaccgcccatgatgctcatcaagaacacgcctgtgcccggaaatatcaccagcttctcggacgtgcccgtcagcagcttcatcacccagtacagcaccgggcaggtcaccgtggagatggagtgggagctcaagaaggaaaactccaagaggtggaacccagagatccagtacacaaacaactacaacgacccccagtttgtggactttgccccggacagcaccggggaatacagaagcaccagacctatcggaacccgataccttacccgacccctttaa

SEQ ID NO: 31 - DNA, 1767 bp, synthetic construct
  source 1..1767: mol_type = other DNA
acggcccctaccggaaagcggatagacgaccactttccaaaaagaaagaaggctcggaccgaagaggactccaagccttccacctcgtcagacgccgaagctggacccagcggatcccagcagctgcaaatcccagcccaaccagcctcaagtttgggagctgatacaatgtctgcgggaggtggcggcccattgggcgacaataaccaaggtgccgatggagtgggcaatgcctcgggagattggcattgcgattccacgtggatgggggacagagtcgtcaccaagtccacccgaacctgggtgctgcccagctacaacaaccaccagtaccgagagatcaaaagcggctccgtcgacggaagcaacgccaacgcctactttggatacagcaccccctgggggtactttgactttaaccgcttccacagccactggagcccccgagactggcaaagactcatcaacaactactggggcttcagaccccggtccctcagagtcaaaatcttcaacattcaagtcaaagaggtcacggtgcaggactccaccaccaccatcgccaacaacctcacctccaccgtccaagtgtttacggacgacgactaccagctgccctacgtcgtcggcaacgggaccgagggatgcctgccggccttccctccgcaggtctttacgctgccgcagtacggttacgcgacgctgaaccgcgacaacacagaaaatcccaccgagaggagcagcttcttctgcctagagtactttcccagcaagatgctgagaacgggcaacaactttgagtttacctacaactttgaggaggtgcccttccactccagcttcgctcccagtcagaacctcttcaagctggccaacccgctggtggaccagtacttgtaccgcttcgtgagcacaaataacactggcggagtccagttcaacaagaacctggccgggagatacgccaacacctacaaaaactggttcccggggcccatgggccgaacccagggctggaacctgggctccggggtcaaccgcgccagtgtcagcgccttcgccacgaccaataggatggagctcgagggcgcgagttaccaggtgcccccgcagccgaacggcatgaccaacaacctccagggcagcaacacctatgccctggagaacactatgatcttcaacagccagccggcgaacccgggcaccaccgccacgtacctcgagggcaacatgctcatcaccagcgagagcgagacgcagccggtgaaccgcgtggcgtacaacgtcggcgggcagatggccaccaacaaccagagctccaccactgcccccgcgaccggcacgtacaacctccaggaaatcgtgcccggcagcgtgtggatggagagggacgtgtacctccaaggacccatctgggccaagatcccagaggtcggggcgcactttcacccctctccggccatgggcggattcggactcaaacacccaccgcccatgatgctcatcaagaacacgcctgtgcccggaaatatcaccagcttctcggacgtgcccgtcagcagcttcatcacccagtacagcaccgggcaggtcaccgtggagatggagtgggagctcaagaaggaaaactccaagaggtggaacccagagatccagtacacaaacaactacaacgacccccagtttgtggactttgccccggacagcaccggggaatacagaaccaccagacctatcggaacccgataccttacccgacccctttaa

SEQ ID NO: 32 - DNA, 1767 bp, synthetic construct
  source 1..1767: mol_type = other DNA
acggcccctaccggaaagcggatagacgaccactttccaaaaagaaagaaggctcggaccgaagaggactccaagccttccacctcgtcagacgccgaagctggacccagcggatcccagcagctgcaaatcccagcccaaccagcctcaagtttgggagctgatacaatgtctgcgggaggtggcggcccattgggcgacaataaccaaggtgccgatggagtgggcaatgcctcgggagattggcattgcgattccacgtggatgggggacagagtcgtcaccaagtccacccgaacctgggtgctgcccagctacaacaaccaccagtaccgagagatcaaaagcggctccgtcgacggaagcaacgccaacgcctactttggatacagcaccccctgggggtactttgactttaaccgcttccacagccactggagcccccgagactggcaaagactcatcaacaactactggggcttcagaccccggtccctcagagtcaaaatcttcaacattcaagtcaaagaggtcacggtgcaggactccaccaccaccatcgccaacaacctcacctccaccgtccaagtgtttacggacgacgactaccagctgccctacgtcgtcggcaacgggaccgagggatgcctgccggccttccctccgcaggtctttacgctgccgcagtacggttacgcgacgctgaaccgcgacaacacagaaaatcccaccgagaggagcagcttcttctgcctagagtactttcccagcaagatgctgagaacgggcaacaactttgagtttacctacaactttgaggaggtgcccttccactccagcttcgctcccagtcagaacctcttcaagctggccaacccgctggtggaccagtacttgtaccgcttcgtgagcacaaataacactggcggagtccagttcaacaagaacctggccgggagatacgccaacacctacaaaaactggttcccggggcccatgggccgaacccagggctggaacctgggctccggggtcaaccgcgccagtgtcagcgccttcgccacgaccaataggatggagctcgagggcgcgagttaccaggtgcccccgcagccgaacggcatgaccaacaacctccagggcagcaacacctatgccctggagaacactatgatcttcaacagccagccggcgaacccgggcaccaccgccacgtacctcgagggcaacatgctcatcaccagcgagagcgagacgcagccggtgaaccgcgtggcgtacaacgtcggcgggcagatggccaccaacaaccagagctccaccactgcccccgcgaccggcacgtacaacctccaggaaatcgtgcccggcagcgtgtggatggagagggacgtgtacctccaaggacccatctgggccaagatcccagaggtcggggcgcactttcacccctctccggccatgggcggattcggactcaaacacccaccgcccatgatgctcatcaagaacacgcctgtgcccggaaatatcaccagcttctcggacgtgcccgtcagcagcttcatcacccagtacagcaccgggcaggtcaccgtggagatggagtgggagctcaagaaggaaaactccaagaggtggaacccagagatccagtacacaaacaactacaacgacccccagtttgtggactttgccccggacagcaccggggaatacagaagcaccagacctatcggaacccgataccttacccgacccctttaa

SEQ ID NO: 33 - protein, 532 aa, Adeno-associated dependoparvovirus B
MSAGGGGPLGDNNQGADGVGNASGDWHCDSTWMGDRVVTKSTRTWVLPSYNNHQYREIKSGSVDGSNANAYFGYSTPWGYFDFNRFHSHWSPRDWQRLINNYWGFRPRSLRVKIFNIQVKEVTVQDSTTTIANNLTSTVQVFTDDDYQLPYVVGNGTEGCLPAFPPQVFTLPQYGYATLNRDNTENPTERSSFFCLEYFPSKMLRTGNNFEFTYNFEEVPFHSSFAPSQNLFKLANPLVDQYLYRFVSTNNTGGVQFNKNLAGRYANTYKNWFPGPMGRTQGWNLGSGVNRASVSAFATTNRMELEGASYQVPPQPNGMTNNLQGSNTYALENTMIFNSQPANPGTTATYLEGNMLITSESETQPVNRVAYNVGGQMATNNQSSTTAPATGTYNLQEIVPGSVWMERDVYLQGPIWAKIPETGAHFHPSPAMGGFGLKHPPPMMLIKNTPVPGNITSFSDVPVSSFITQYSTGQVTVEMEWELKKENSKRWNPEIQYTNNYNDPQFVDFAPDSTGEYRTTRPIGTRYLTRPL

SEQ ID NO: 34 - protein, 532 aa, synthetic construct
MSAGGGGPLGDNNQGADGVGNASGDWHCDSTWMGDRVVTKSTRTWVLPSYNNHQYREIKSGSVDGSNANAYFGYSTPWGYFDFNRFHSHWSPRDWQRLINNYWGFRPRSLRVKIFNIQVKEVTVQDSTTTIANNLTSTVQVFTDDDYQLPYVVGNGTEGCLPAFPPQVFTLPQYGYATLNRDNTENPTERSSFFCLEYFPSKMLRTGNNFEFTYNFEEVPFHSSFAPSQNLFKLANPLVDQYLYRFVSTNNTGGVQFNKNLAGRYANTYKNWFPGPMGRTQGWNLGSGVNRASVSAFATTNRMELEGASYQVPPQPNGMTNNLQGSNTYALENTMIFNSQPANPGTTATYLEGNMLITSESETQPVNRVAYNVGGQMATNNQSSTTAPATGTYNLQEIVPGSVWMERDVYLQGPIWAKIPETGAHFHPSPAMGGFGLKHPPPMMLIKNTPVPGNITSFSDVPVSSFITQYSTGQVTVEMEWELKKENSKRWNPEIQYTNNYNDPQFVDFAPDSTGEYRSTRPIGTRYLTRPL

SEQ ID NO: 35 - protein, 532 aa, synthetic construct
MSAGGGGPLGDNNQGADGVGNASGDWHCDSTWMVDRVVTKSTRTWVLPSYNNHQYREIKSGSVDGSNANAYFGYSTPWGYFDFNRFHSHWSPRDWQRLINNYWGFRPRSLRVKIFNIQVKEVTVQDSTTTIANNLTSTVQVFTDDDYQLPYVVGNGTEGCLPAFPPQVFTLPQYGYATLNRDNTENPTERSSFFCLEYFPSKMLRTGNNFEFTYNFEEVPFHSSFAPSQNLFKLANPLVDQYLYRFVSTNNTGGVQFNKNLAGRYANTYKNWFPGPMGRTQGWNLGSGVNRASVSAFATTNRMELEGASYQVPPQPNGMTNNLQGSNTYALENTMIFNSQPANPGTTATYLEGNMLITSESETQPVNRVAYNVGGQMATNNQSSTTAPATGTYNLQEIVPGSVWMERDVYLQGPIWAKIPETGAHFHPSPAMGGFGLKHPPPMMLIKNTPVPGNITSFSDVPVSSFITQYSTGQVTVEMEWELKKENSKRWNPEIQYTNNYNDPQFVDFAPDSTGEYRTTRPIGTRYLTRPL

SEQ ID NO: 36 - protein, 532 aa, synthetic construct
MSAGGGGPLGDNNQGADGVGNASGDWHCDSTWMVDRVVTKSTRTWVLPSYNNHQYREIKSGSVDGSNANAYFGYSTPWGYFDFNRFHSHWSPRDWQRLINNYWGFRPRSLRVKIFNIQVKEVTVQDSTTTIANNLTSTVQVFTDDDYQLPYVVGNGTEGCLPAFPPQVFTLPQYGYATLNRDNTENPTERSSFFCLEYFPSKMLRTGNNFEFTYNFEEVPFHSSFAPSQNLFKLANPLVDQYLYRFVSTNNTGGVQFNKNLAGRYANTYKNWFPGPMGRTQGWNLGSGVNRASVSAFATTNRMELEGASYQVPPQPNGMTNNLQGSNTYALENTMIFNSQPANPGTTATYLEGNMLITSESETQPVNRVAYNVGGQMATNNQSSTTAPATGTYNLQEIVPGSVWMERDVYLQGPIWAKIPETGAHFHPSPAMGGFGLKHPPPMMLIKNTPVPGNITSFSDVPVSSFITQYSTGQVTVEMEWELKKENSKRWNPEIQYTNNYNDPQFVDFAPDSTGEYRSTRPIGTRYLTRPL

SEQ ID NO: 37 - protein, 532 aa, synthetic construct
MSAGGGGPLGDNNQGADGVGNASGDWHCDSTWMGDRVVTKSTRTWVLPSYNNHQYREIKSGSVDGSNANAYFGYSTPWGYFDFNRFHSHWSPRDWQRLINNYWGFRPRSLRVKIFNIQVKEVTVQDSTTTIANNLTSTVQVFTDDDYQLPYVVGNGTEGCLPAFPPQVFTLPQYGYATLNRDNTENPTERSSFFCLEYFPSKMLRTGNNFEFTYNFEEVPFHSSFAPSQNLFKLANPLVDQYLYRFVSTNNTGGVQFNKNLAGRYANTYKNWFPGPMGRTQGWNLGSGVNRASVSAFATTNRMELEGASYQVPPQPNGMTNNLQGSNTYALENTMIFNSQPANPGTTATYLEGNMLITSESETQPVNRVAYNVGGQMATNNQSSTTAPATGTYNLQEIVPGSVWMERDVYLQGPIWAKIPEAGAHFHPSPAMGGFGLKHPPPMMLIKNTPVPGNITSFSDVPVSSFITQYSTGQVTVEMEWELKKENSKRWNPEIQYTNNYNDPQFVDFAPDSTGEYRTTRPIGTRYLTRPL

SEQ ID NO: 38 - protein, 532 aa, synthetic construct
MSAGGGGPLGDNNQGADGVGNASGDWHCDSTWMGDRVVTKSTRTWVLPSYNNHQYREIKSGSVDGSNANAYFGYSTPWGYFDFNRFHSHWSPRDWQRLINNYWGFRPRSLRVKIFNIQVKEVTVQDSTTTIANNLTSTVQVFTDDDYQLPYVVGNGTEGCLPAFPPQVFTLPQYGYATLNRDNTENPTERSSFFCLEYFPSKMLRTGNNFEFTYNFEEVPFHSSFAPSQNLFKLANPLVDQYLYRFVSTNNTGGVQFNKNLAGRYANTYKNWFPGPMGRTQGWNLGSGVNRASVSAFATTNRMELEGASYQVPPQPNGMTNNLQGSNTYALENTMIFNSQPANPGTTATYLEGNMLITSESETQPVNRVAYNVGGQMATNNQSSTTAPATGTYNLQEIVPGSVWMERDVYLQGPIWAKIPEAGAHFHPSPAMGGFGLKHPPPMMLIKNTPVPGNITSFSDVPVSSFITQYSTGQVTVEMEWELKKENSKRWNPEIQYTNNYNDPQFVDFAPDSTGEYRSTRPIGTRYLTRPL

SEQ ID NO: 39 - protein, 532 aa, synthetic construct
MSAGGGGPLGDNNQGADGVGNASGDWHCDSTWMGDRVVTKSTRTWVLPSYNNHQYREIKSGSVDGSNANAYFGYSTPWGYFDFNRFHSHWSPRDWQRLINNYWGFRPRSLRVKIFNIQVKEVTVQDSTTTIANNLTSTVQVFTDDDYQLPYVVGNGTEGCLPAFPPQVFTLPQYGYATLNRDNTENPTERSSFFCLEYFPSKMLRTGNNFEFTYNFEEVPFHSSFAPSQNLFKLANPLVDQYLYRFVSTNNTGGVQFNKNLAGRYANTYKNWFPGPMGRTQGWNLGSGVNRASVSAFATTNRMELEGASYQVPPQPNGMTNNLQGSNTYALENTMIFNSQPANPGTTATYLEGNMLITSESETQPVNRVAYNVGGQMATNNQSSTTAPATGTYNLQEIVPGSVWMERDVYLQGPIWAKIPEVGAHFHPSPAMGGFGLKHPPPMMLIKNTPVPGNITSFSDVPVSSFITQYSTGQVTVEMEWELKKENSKRWNPEIQYTNNYNDPQFVDFAPDSTGEYRTTRPIGTRYLTRPL

SEQ ID NO: 40 - protein, 532 aa, synthetic construct
MSAGGGGPLGDNNQGADGVGNASGDWHCDSTWMGDRVVTKSTRTWVLPSYNNHQYREIKSGSVDGSNANAYFGYSTPWGYFDFNRFHSHWSPRDWQRLINNYWGFRPRSLRVKIFNIQVKEVTVQDSTTTIANNLTSTVQVFTDDDYQLPYVVGNGTEGCLPAFPPQVFTLPQYGYATLNRDNTENPTERSSFFCLEYFPSKMLRTGNNFEFTYNFEEVPFHSSFAPSQNLFKLANPLVDQYLYRFVSTNNTGGVQFNKNLAGRYANTYKNWFPGPMGRTQGWNLGSGVNRASVSAFATTNRMELEGASYQVPPQPNGMTNNLQGSNTYALENTMIFNSQPANPGTTATYLEGNMLITSESETQPVNRVAYNVGGQMATNNQSSTTAPATGTYNLQEIVPGSVWMERDVYLQGPIWAKIPEVGAHFHPSPAMGGFGLKHPPPMMLIKNTPVPGNITSFSDVPVSSFITQYSTGQVTVEMEWELKKENSKRWNPEIQYTNNYNDPQFVDFAPDSTGEYRSTRPIGTRYLTRPL

SEQ ID NO: 41 - DNA, 1599 bp, Adeno-associated dependoparvovirus B
  source 1..1599: mol_type = genomic DNA
atgtctgcgggaggtggcggcccattgggcgacaataaccaaggtgccgatggagtgggcaatgcctcgggagattggcattgcgattccacgtggatgggggacagagtcgtcaccaagtccacccgaacctgggtgctgcccagctacaacaaccaccagtaccgagagatcaaaagcggctccgtcgacggaagcaacgccaacgcctactttggatacagcaccccctgggggtactttgactttaaccgcttccacagccactggagcccccgagactggcaaagactcatcaacaactactggggcttcagaccccggtccctcagagtcaaaatcttcaacattcaagtcaaagaggtcacggtgcaggactccaccaccaccatcgccaacaacctcacctccaccgtccaagtgtttacggacgacgactaccagctgccctacgtcgtcggcaacgggaccgagggatgcctgccggccttccctccgcaggtctttacgctgccgcagtacggttacgcgacgctgaaccgcgacaacacagaaaatcccaccgagaggagcagcttcttctgcctagagtactttcccagcaagatgctgagaacgggcaacaactttgagtttacctacaactttgaggaggtgcccttccactccagcttcgctcccagtcagaacctcttcaagctggccaacccgctggtggaccagtacttgtaccgcttcgtgagcacaaataacactggcggagtccagttcaacaagaacctggccgggagatacgccaacacctacaaaaactggttcccggggcccatgggccgaacccagggctggaacctgggctccggggtcaaccgcgccagtgtcagcgccttcgccacgaccaataggatggagctcgagggcgcgagttaccaggtgcccccgcagccgaacggcatgaccaacaacctccagggcagcaacacctatgccctggagaacactatgatcttcaacagccagccggcgaacccgggcaccaccgccacgtacctcgagggcaacatgctcatcaccagcgagagcgagacgcagccggtgaaccgcgtggcgtacaacgtcggcgggcagatggccaccaacaaccagagctccaccactgcccccgcgaccggcacgtacaacctccaggaaatcgtgcccggcagcgtgtggatggagagggacgtgtacctccaaggacccatctgggccaagatcccagagacgggggcgcactttcacccctctccggccatgggcggattcggactcaaacacccaccgcccatgatgctcatcaagaacacgcctgtgcccggaaatatcaccagcttctcggacgtgcccgtcagcagcttcatcacccagtacagcaccgggcaggtcaccgtggagatggagtgggagctcaagaaggaaaactccaagaggtggaacccagagatccagtacacaaacaactacaacgacccccagtttgtggactttgccccggacagcaccggggaatacagaaccaccagacctatcggaacccgataccttacccgacccctttaa

SEQ ID NO: 42 - DNA, 1599 bp, synthetic construct
  source 1..1599: mol_type = other DNA
atgtctgcgggaggtggcggcccattgggcgacaataaccaaggtgccgatggagtgggcaatgcctcgggagattggcattgcgattccacgtggatgggggacagagtcgtcaccaagtccacccgaacctgggtgctgcccagctacaacaaccaccagtaccgagagatcaaaagcggctccgtcgacggaagcaacgccaacgcctactttggatacagcaccccctgggggtactttgactttaaccgcttccacagccactggagcccccgagactggcaaagactcatcaacaactactggggcttcagaccccggtccctcagagtcaaaatcttcaacattcaagtcaaagaggtcacggtgcaggactccaccaccaccatcgccaacaacctcacctccaccgtccaagtgtttacggacgacgactaccagctgccctacgtcgtcggcaacgggaccgagggatgcctgccggccttccctccgcaggtctttacgctgccgcagtacggttacgcgacgctgaaccgcgacaacacagaaaatcccaccgagaggagcagcttcttctgcctagagtactttcccagcaagatgctgagaacgggcaacaactttgagtttacctacaactttgaggaggtgcccttccactccagcttcgctcccagtcagaacctcttcaagctggccaacccgctggtggaccagtacttgtaccgcttcgtgagcacaaataacactggcggagtccagttcaacaagaacctggccgggagatacgccaacacctacaaaaactggttcccggggcccatgggccgaacccagggctggaacctgggctccggggtcaaccgcgccagtgtcagcgccttcgccacgaccaataggatggagctcgagggcgcgagttaccaggtgcccccgcagccgaacggcatgaccaacaacctccagggcagcaacacctatgccctggagaacactatgatcttcaacagccagccggcgaacccgggcaccaccgccacgtacctcgagggcaacatgctcatcaccagcgagagcgagacgcagccggtgaaccgcgtggcgtacaacgtcggcgggcagatggccaccaacaaccagagctccaccactgcccccgcgaccggcacgtacaacctccaggaaatcgtgcccggcagcgtgtggatggagagggacgtgtacctccaaggacccatctgggccaagatcccagagacgggggcgcactttcacccctctccggccatgggcggattcggactcaaacacccaccgcccatgatgctcatcaagaacacgcctgtgcccggaaatatcaccagcttctcggacgtgcccgtcagcagcttcatcacccagtacagcaccgggcaggtcaccgtggagatggagtgggagctcaagaaggaaaactccaagaggtggaacccagagatccagtacacaaacaactacaacgacccccagtttgtggactttgccccggacagcaccggggaatacagaagcaccagacctatcggaacccgataccttacccgacccctttaa

SEQ ID NO: 43 - DNA, 1599 bp, synthetic construct
  source 1..1599: mol_type = other DNA
atgtctgcgggaggtggcggcccattgggcgacaataaccaaggtgccgatggagtgggcaatgcctcgggagattggcattgcgattccacgtggatggtcgacagagtcgtcaccaagtccacccgaacctgggtgctgcccagctacaacaaccaccagtaccgagagatcaaaagcggctccgtcgacggaagcaacgccaacgcctactttggatacagcaccccctgggggtactttgactttaaccgcttccacagccactggagcccccgagactggcaaagactcatcaacaactactggggcttcagaccccggtccctcagagtcaaaatcttcaacattcaagtcaaagaggtcacggtgcaggactccaccaccaccatcgccaacaacctcacctccaccgtccaagtgtttacggacgacgactaccagctgccctacgtcgtcggcaacgggaccgagggatgcctgccggccttccctccgcaggtctttacgctgccgcagtacggttacgcgacgctgaaccgcgacaacacagaaaatcccaccgagaggagcagcttcttctgcctagagtactttcccagcaagatgctgagaacgggcaacaactttgagtttacctacaactttgaggaggtgcccttccactccagcttcgctcccagtcagaacctcttcaagctggccaacccgctggtggaccagtacttgtaccgcttcgtgagcacaaataacactggcggagtccagttcaacaagaacctggccgggagatacgccaacacctacaaaaactggttcccggggcccatgggccgaacccagggctggaacctgggctccggggtcaaccgcgccagtgtcagcgccttcgccacgaccaataggatggagctcgagggcgcgagttaccaggtgcccccgcagccgaacggcatgaccaacaacctccagggcagcaacacctatgccctggagaacactatgatcttcaacagccagccggcgaacccgggcaccaccgccacgtacctcgagggcaacatgctcatcaccagcgagagcgagacgcagccggtgaaccgcgtggcgtacaacgtcggcgggcagatggccaccaacaaccagagctccaccactgcccccgcgaccggcacgtacaacctccaggaaatcgtgcccggcagcgtgtggatggagagggacgtgtacctccaaggacccatctgggccaagatcccagagacgggggcgcactttcacccctctccggccatgggcggattcggactcaaacacccaccgcccatgatgctcatcaagaacacgcctgtgcccggaaatatcaccagcttctcggacgtgcccgtcagcagcttcatcacccagtacagcaccgggcaggtcaccgtggagatggagtgggagctcaagaaggaaaactccaagaggtggaacccagagatccagtacacaaacaactacaacgacccccagtttgtggactttgccccggacagcaccggggaatacagaaccaccagacctatcggaacccgataccttacccgacccctttaa

SEQ ID NO: 44 - DNA, 1599 bp, synthetic construct
  source 1..1599: mol_type = other DNA
atgtctgcgggaggtggcggcccattgggcgacaataaccaaggtgccgatggagtgggcaatgcctcgggagattggcattgcgattccacgtggatggtcgacagagtcgtcaccaagtccacccgaacctgggtgctgcccagctacaacaaccaccagtaccgagagatcaaaagcggctccgtcgacggaagcaacgccaacgcctactttggatacagcaccccctgggggtactttgactttaaccgcttccacagccactggagcccccgagactggcaaagactcatcaacaactactggggcttcagaccccggtccctcagagtcaaaatcttcaacattcaagtcaaagaggtcacggtgcaggactccaccaccaccatcgccaacaacctcacctccaccgtccaagtgtttacggacgacgactaccagctgccctacgtcgtcggcaacgggaccgagggatgcctgccggccttccctccgcaggtctttacgctgccgcagtacggttacgcgacgctgaaccgcgacaacacagaaaatcccaccgagaggagcagcttcttctgcctagagtactttcccagcaagatgctgagaacgggcaacaactttgagtttacctacaactttgaggaggtgcccttccactccagcttcgctcccagtcagaacctcttcaagctggccaacccgctggtggaccagtacttgtaccgcttcgtgagcacaaataacactggcggagtccagttcaacaagaacctggccgggagatacgccaacacctacaaaaactggttcccggggcccatgggccgaacccagggctggaacctgggctccggggtcaaccgcgccagtgtcagcgccttcgccacgaccaataggatggagctcgagggcgcgagttaccaggtgcccccgcagccgaacggcatgaccaacaacctccagggcagcaacacctatgccctggagaacactatgatcttcaacagccagccggcgaacccgggcaccaccgccacgtacctcgagggcaacatgctcatcaccagcgagagcgagacgcagccggtgaaccgcgtggcgtacaacgtcggcgggcagatggccaccaacaaccagagctccaccactgcccccgcgaccggcacgtacaacctccaggaaatcgtgcccggcagcgtgtggatggagagggacgtgtacctccaaggacccatctgggccaagatcccagagacgggggcgcactttcacccctctccggccatgggcggattcggactcaaacacccaccgcccatgatgctcatcaagaacacgcctgtgcccggaaatatcaccagcttctcggacgtgcccgtcagcagcttcatcacccagtacagcaccgggcaggtcaccgtggagatggagtgggagctcaagaaggaaaactccaagaggtggaacccagagatccagtacacaaacaactacaacgacccccagtttgtggactttgccccggacagcaccggggaatacagaagcaccagacctatcggaacccgataccttacccgacccctttaa

SEQ ID NO: 45 - DNA, 1599 bp, synthetic construct
  source 1..1599: mol_type = other DNA
atgtctgcgggaggtggcggcccattgggcgacaataaccaaggtgccgatggagtgggcaatgcctcgggagattggcattgcgattccacgtggatgggggacagagtcgtcaccaagtccacccgaacctgggtgctgcccagctacaacaaccaccagtaccgagagatcaaaagcggctccgtcgacggaagcaacgccaacgcctactttggatacagcaccccctgggggtactttgactttaaccgcttccacagccactggagcccccgagactggcaaagactcatcaacaactactggggcttcagaccccggtccctcagagtcaaaatcttcaacattcaagtcaaagaggtcacggtgcaggactccaccaccaccatcgccaacaacctcacctccaccgtccaagtgtttacggacgacgactaccagctgccctacgtcgtcggcaacgggaccgagggatgcctgccggccttccctccgcaggtctttacgctgccgcagtacggttacgcgacgctgaaccgcgacaacacagaaaatcccaccgagaggagcagcttcttctgcctagagtactttcccagcaagatgctgagaacgggcaacaactttgagtttacctacaactttgaggaggtgcccttccactccagcttcgctcccagtcagaacctcttcaagctggccaacccgctggtggaccagtacttgtaccgcttcgtgagcacaaataacactggcggagtccagttcaacaagaacctggccgggagatacgccaacacctacaaaaactggttcccggggcccatgggccgaacccagggctggaacctgggctccggggtcaaccgcgccagtgtcagcgccttcgccacgaccaataggatggagctcgagggcgcgagttaccaggtgcccccgcagccgaacggcatgaccaacaacctccagggcagcaacacctatgccctggagaacactatgatcttcaacagccagccggcgaacccgggcaccaccgccacgtacctcgagggcaacatgctcatcaccagcgagagcgagacgcagccggtgaaccgcgtggcgtacaacgtcggcgggcagatggccaccaacaaccagagctccaccactgcccccgcgaccggcacgtacaacctccaggaaatcgtgcccggcagcgtgtggatggagagggacgtgtacctccaaggacccatctgggccaagatcccagaggccggggcgcactttcacccctctccggccatgggcggattcggactcaaacacccaccgcccatgatgctcatcaagaacacgcctgtgcccggaaatatcaccagcttctcggacgtgcccgtcagcagcttcatcacccagtacagcaccgggcaggtcaccgtggagatggagtgggagctcaagaaggaaaactccaagaggtggaacccagagatccagtacacaaacaactacaacgacccccagtttgtggactttgccccggacagcaccggggaatacagaaccaccagacctatcggaacccgataccttacccgacccctttaa

SEQ ID NO: 46 - DNA, 1599 bp, synthetic construct
  source 1..1599: mol_type = other DNA
atgtctgcgggaggtggcggcccattgggcgacaataaccaaggtgccgatggagtgggcaatgcctcgggagattggcattgcgattccacgtggatgggggacagagtcgtcaccaagtccacccgaacctgggtgctgcccagctacaacaaccaccagtaccgagagatcaaaagcggctccgtcgacggaagcaacgccaacgcctactttggatacagcaccccctgggggtactttgactttaaccgcttccacagccactggagcccccgagactggcaaagactcatcaacaactactggggcttcagaccccggtccctcagagtcaaaatcttcaacattcaagtcaaagaggtcacggtgcaggactccaccaccaccatcgccaacaacctcacctccaccgtccaagtgtttacggacgacgactaccagctgccctacgtcgtcggcaacgggaccgagggatgcctgccggccttccctccgcaggtctttacgctgccgcagtacggttacgcgacgctgaaccgcgacaacacagaaaatcccaccgagaggagcagcttcttctgcctagagtactttcccagcaagatgctgagaacgggcaacaactttgagtttacctacaactttgaggaggtgcccttccactccagcttcgctcccagtcagaacctcttcaagctggccaacccgctggtggaccagtacttgtaccgcttcgtgagcacaaataacactggcggagtccagttcaacaagaacctggccgggagatacgccaacacctacaaaaactggttcccggggcccatgggccgaacccagggctggaacctgggctccggggtcaaccgcgccagtgtcagcgccttcgccacgaccaataggatggagctcgagggcgcgagttaccaggtgcccccgcagccgaacggcatgaccaacaacctccagggcagcaacacctatgccctggagaacactatgatcttcaacagccagccggcgaacccgggcaccaccgccacgtacctcgagggcaacatgctcatcaccagcgagagcgagacgcagccggtgaaccgcgtggcgtacaacgtcggcgggcagatggccaccaacaaccagagctccaccactgcccccgcgaccggcacgtacaacctccaggaaatcgtgcccggcagcgtgtggatggagagggacgtgtacctccaaggacccatctgggccaagatcccagaggccggggcgcactttcacccctctccggccatgggcggattcggactcaaacacccaccgcccatgatgctcatcaagaacacgcctgtgcccggaaatatcaccagcttctcggacgtgcccgtcagcagcttcatcacccagtacagcaccgggcaggtcaccgtggagatggagtgggagctcaagaaggaaaactccaagaggtggaacccagagatccagtacacaaacaactacaacgacccccagtttgtggactttgccccggacagcaccggggaatacagaagcaccagacctatcggaacccgataccttacccgacccctttaa

SEQ ID NO: 47 - DNA, 1599 bp, synthetic construct
  source 1..1599: mol_type = other DNA
atgtctgcgggaggtggcggcccattgggcgacaataaccaaggtgccgatggagtgggcaatgcctcgggagattggcattgcgattccacgtggatgggggacagagtcgtcaccaagtccacccgaacctgggtgctgcccagctacaacaaccaccagtaccgagagatcaaaagcggctccgtcgacggaagcaacgccaacgcctactttggatacagcaccccctgggggtactttgactttaaccgcttccacagccactggagcccccgagactggcaaagactcatcaacaactactggggcttcagaccccggtccctcagagtcaaaatcttcaacattcaagtcaaagaggtcacggtgcaggactccaccaccaccatcgccaacaacctcacctccaccgtccaagtgtttacggacgacgactaccagctgccctacgtcgtcggcaacgggaccgagggatgcctgccggccttccctccgcaggtctttacgctgccgcagtacggttacgcgacgctgaaccgcgacaacacagaaaatcccaccgagaggagcagcttcttctgcctagagtactttcccagcaagatgctgagaacgggcaacaactttgagtttacctacaactttgaggaggtgcccttccactccagcttcgctcccagtcagaacctcttcaagctggccaacccgctggtggaccagtacttgtaccgcttcgtgagcacaaataacactggcggagtccagttcaacaagaacctggccgggagatacgccaacacctacaaaaactggttcccggggcccatgggccgaacccagggctggaacctgggctccggggtcaaccgcgccagtgtcagcgccttcgccacgaccaataggatggagctcgagggcgcgagttaccaggtgcccccgcagccgaacggcatgaccaacaacctccagggcagcaacacctatgccctggagaacactatgatcttcaacagccagccggcgaacccgggcaccaccgccacgtacctcgagggcaacatgctcatcaccagcgagagcgagacgcagccggtgaaccgcgtggcgtacaacgtcggcgggcagatggccaccaacaaccagagctccaccactgcccccgcgaccggcacgtacaacctccaggaaatcgtgcccggcagcgtgtggatggagagggacgtgtacctccaaggacccatctgggccaagatcccagaggtcggggcgcactttcacccctctccggccatgggcggattcggactcaaacacccaccgcccatgatgctcatcaagaacacgcctgtgcccggaaatatcaccagcttctcggacgtgcccgtcagcagcttcatcacccagtacagcaccgggcaggtcaccgtggagatggagtgggagctcaagaaggaaaactccaagaggtggaacccagagatccagtacacaaacaactacaacgacccccagtttgtggactttgccccggacagcaccggggaatacagaaccaccagacctatcggaacccgataccttacccgacccctttaa

SEQ ID NO: 48 - DNA, 1599 bp, synthetic construct
  source 1..1599: mol_type = other DNA
atgtctgcgggaggtggcggcccattgggcgacaataaccaaggtgccgatggagtgggcaatgcctcgggagattggcattgcgattccacgtggatgggggacagagtcgtcaccaagtccacccgaacctgggtgctgcccagctacaacaaccaccagtaccgagagatcaaaagcggctccgtcgacggaagcaacgccaacgcctactttggatacagcaccccctgggggtactttgactttaaccgcttccacagccactggagcccccgagactggcaaagactcatcaacaactactggggcttcagaccccggtccctcagagtcaaaatcttcaacattcaagtcaaagaggtcacggtgcaggactccaccaccaccatcgccaacaacctcacctccaccgtccaagtgtttacggacgacgactaccagctgccctacgtcgtcggcaacgggaccgagggatgcctgccggccttccctccgcaggtctttacgctgccgcagtacggttacgcgacgctgaaccgcgacaacacagaaaatcccaccgagaggagcagcttcttctgcctagagtactttcccagcaagatgctgagaacgggcaacaactttgagtttacctacaactttgaggaggtgcccttccactccagcttcgctcccagtcagaacctcttcaagctggccaacccgctggtggaccagtacttgtaccgcttcgtgagcacaaataacactggcggagtccagttcaacaagaacctggccgggagatacgccaacacctacaaaaactggttcccggggcccatgggccgaacccagggctggaacctgggctccggggtcaaccgcgccagtgtcagcgccttcgccacgaccaataggatggagctcgagggcgcgagttaccaggtgcccccgcagccgaacggcatgaccaacaacctccagggcagcaacacctatgccctggagaacactatgatcttcaacagccagccggcgaacccgggcaccaccgccacgtacctcgagggcaacatgctcatcaccagcgagagcgagacgcagccggtgaaccgcgtggcgtacaacgtcggcgggcagatggccaccaacaaccagagctccaccactgcccccgcgaccggcacgtacaacctccaggaaatcgtgcccggcagcgtgtggatggagagggacgtgtacctccaaggacccatctgggccaagatcccagaggtcggggcgcactttcacccctctccggccatgggcggattcggactcaaacacccaccgcccatgatgctcatcaagaacacgcctgtgcccggaaatatcaccagcttctcggacgtgcccgtcagcagcttcatcacccagtacagcaccgggcaggtcaccgtggagatggagtgggagctcaagaaggaaaactccaagaggtggaacccagagatccagtacacaaacaactacaacgacccccagtttgtggactttgccccggacagcaccggggaatacagaagcaccagacctatcggaacccgataccttacccgacccctttaa